European Patent Specification EP 3 405 481 B1, published January 18, 2023. Title: Chimeric Antigen Receptors Targeting Epidermal Growth Factor Receptor Variant III. Applicant: PFIZER INC. Wong, Oi Kwan Chou, Joyce C Dusseaux, Mathilde Brunnhilde C Smith, Julianne C. Application PCT/IB2017/050108. The sequence listing filed with the application follows.

SEQUENCE LISTING (277 sequences)

SEQ ID NO: 1 - protein, 115 aa, Artificial Sequence
  Synthetic Construct
EVQLQQSGPELVKPGASVKISCKTSGYTFTDYTLHWVKQSHVKSLEWIGGIDPINGGTTYNQKFKGKATLTVDKSSSTAYMELRSLTSEDSAVYYCARGEAMDSWGQGTSVTVSS

SEQ ID NO: 2 - protein, 112 aa, Artificial Sequence
  Synthetic Construct
DVVMTQTPLTLSVTIGQPASISCKSSQSLLYSNGKTYLNWLLQRPGQSPKRLIYLVSKLDSGVPDRFTGSGSGTDFTLKISRVEAEDLGFYYCVQDTHFPLTFGAGTKLELK

SEQ ID NO: 3 - protein, 115 aa, Artificial Sequence
  Synthetic Construct
QVQLVQSGAEVKKPGASVKVSCKASGYTFTDYTLHWVRQAPGQGLEWMGGINPINGGTTYNQKFKGRVTMTRDTSTSTVYMELSSLRSEDTAVYYCARGEAMDSWGQGTLVTVSS

SEQ ID NO: 4 - protein, 112 aa, Artificial Sequence
  Synthetic Construct
DVVMTQSPLSLPVTLGQPASISCKSSQSLLYSNGKTYLNWFQQRPGQSPRRLIYLVSKLDSGVPDRFSGSGSGTDFTLKISRVEAEDVGVYYCVQDTHFPLTFGGGTKVEIK

SEQ ID NO: 5 - protein, 115 aa, Artificial Sequence
  Synthetic Construct
QVQLVQSGAEVKKPGASVKVSCKASGYTFTDYTLHWVRQAPGQGLEWMGGIWPITGGTTYNQKFKGRVTMTRDTSTSTVYMELSSLRSEDTAVYYCARGEAQGSWGQGTLVTVSS

SEQ ID NO: 6 - protein, 112 aa, Artificial Sequence
  Synthetic Construct
DVVMTQSPLSLPVTLGQPASISCKSSQSLLYSNGKTYLNWFQQRPGQSPRRLIYQVSKLDSGVPDRFSGSGSGTDFTLKISRVEAEDVGVYYCGQDTHFPLTFGGGTKVEIK

SEQ ID NO: 7 - protein, 115 aa, Artificial Sequence
  Synthetic Construct
QVQLVQSGAEVKKPGASVKVSCKASGYTFTDYTLHWVRQAPGQGLEWMGGIWPITGGTTYNQKFKGRVTMTRDTSTSTVYMELSSLRSEDTAVYYCARGEAEGSWGQGTLVTVSS

SEQ ID NO: 8 - protein, 112 aa, Artificial Sequence
  Synthetic Construct
DVVMTQSPLSLPVTLGQPASISCKSSQSLLYSNDKTYTNWFQQRPGQSPRRLIYEVSKLDVGVPDRFSGSGSGTDFTLKISRVEAEDVGVYYCGQDTHFPLTFGGGTKVEIK

SEQ ID NO: 9 - protein, 121 aa, Artificial Sequence
  Synthetic Construct
QVTLKESGPVLLKPTETLTLTCTVSGFSLSNPRMGVSWIRQPPGKALEWFAHIFSTDEKSLKLSLRSRLTLSKDTSKSQVVLTMTNMAPVDSATYYCARDSSNYEGYFDFWGQGTLVTVSS

SEQ ID NO: 10 - protein, 107 aa, Artificial Sequence
  Synthetic Construct
EVVLTQSPATLSVSPGERATLSCRASQSVRSNLAWYQQKSGQAPRLLIYGSTIRATGVPARFSGSGSGTEFTLTISSLQSEDFAVYYCQQYSDWPFTFGPGTKVDIK

SEQ ID NO: 11 - protein, 121 aa, Artificial Sequence
  Synthetic Construct
QVTLKESGPVLVKPTETLTLTCTVSGFSLSNARMGVSWIRQPPGKALEWLAHIFSTDEKSIRRSLRSRLTLSKDTSKSQVVLTMTNMDPVDTATYFCARDSSNYEGYFDYWGQGTLVTVSS

SEQ ID NO: 12 - protein, 107 aa, Artificial Sequence
  Synthetic Construct
EVVMTQSPATLSVSPGERVTLSCRASQSVSSNFAWYQQRPGQAPRLLLYGATTRATGLPGRFSGSGSGTENILTISSLQSEDFAIYFCQQYKDWPFTFGPGSKVDIK

SEQ ID NO: 13 - protein, 121 aa, Artificial Sequence
  Synthetic Construct
QVTLKESGPVLVKPTETLTLTCTVSGFSLSNARMGVSWIRQPPGKALEWLGHIFSTDEKSYSTSLRGRITISKDTSRGLVVLTLTNMDPVDTATYYCARDSSNYEGYFDFWGPGFLVTVSS

SEQ ID NO: 14 - protein, 107 aa, Artificial Sequence
  Synthetic Construct
EIVMTQSPATLSVSPGERATLSCRVSQSIGANLAWYQQKFGQAPRLLIYGASTRATGIPVRFSGGGSGTEFTLTISSLQSEDFAIYSCQQYIYWPFTFGPGTTVDIK

SEQ ID NO: 15 - protein, 121 aa, Artificial Sequence
  Synthetic Construct
QVTLKESGPVLVKPTETLTLTCTVSGFSLNNARMGVSWIRQPPGKALEWFAHIFSTDEKSFRTSLRSRLTLSKDTSKSQVVLTMTNMDPVDTATYYCARDSSNYEGYFDYWGQGILVTVSS

SEQ ID NO: 16 - protein, 107 aa, Artificial Sequence
  Synthetic Construct
EIVMTQSPATLSVSPGERATLSCRASQSVSNNLAWYQQKPGQAPRLLIYGASTRATGVPARFSGSDSGTEFSLTISSLQSEDFAVYFCQQYKDWPFTFGPGTKVEIK

SEQ ID NO: 17 - protein, 122 aa, Artificial Sequence
  Synthetic Construct
QVTLKESGPVLVKPTETLTLTCTVSGFSLSNVRMGVSWIRQPPGKALEWFAHIFSSDEKSIRRSLRSRLTLSKDTSKSQVVLTMTNMDPVDTATYYCARDSSNYEGYFDFWGQGTLVTVSSN

SEQ ID NO: 18 - protein, 107 aa, Artificial Sequence
  Synthetic Construct
DMVVTQSPATLSVSPGERATLSCRASQSVGSDLAWYQQPPGQSPRLLIYGASTRATGVPARFSGSGSGTDFTLTITSLESEDFAVYYCQQYNDWPFTFGPGTKVDIK

SEQ ID NO: 19 - protein, 121 aa, Artificial Sequence
  Synthetic Construct
QVTLKESGPVLVKPTETLTLTCTVSGFSLSNVRMGVSWIRQPPGKALEWFAHIFSSDEKSIRRSLRSRLTLSKDTSKSQVVLTMTNMDPVDTATYYCARDSSNYEGYFDYWGQGTLVTVSS

SEQ ID NO: 20 - protein, 107 aa, Artificial Sequence
  Synthetic Construct
EMEVTQSPATLSVSPGERATLSCRASQNIGSDLAWYQQQSGQAPRLLISGASTRATGVPTRFSGSGSGTDFTLTITSLQSEDFAVYYCQQYNDWPFTFGPGTKVDIK

SEQ ID NO: 21 - protein, 121 aa, Artificial Sequence
  Synthetic Construct
QVTLKESGPVLVKPTETLTLTCTVSGFSLSNARMGVSWIRQPPGKALEWLAHIFSTDEKSIRRSLRSRLTLSKDTSKSQVVLIMTNMDPVDTATYYCARDSSNYEGYFDYWGQGTLVTVSS

SEQ ID NO: 22 - protein, 107 aa, Artificial Sequence
  Synthetic Construct
EVVMTQSPPNLSVSPGERATLSCRASQSVTSNFAWYQQRPGQSPRLLLYGASTRATGVPGRFSGSGSGTENILTISSLQSEDFAVYFCQQYKDWPFTFGPGSKVDIK

SEQ ID NO: 23 - protein, 121 aa, Artificial Sequence
  Synthetic Construct
QVTLKESGPVLVKPTETLTLTCTVSGFSLSNARMGVSWIRQPPGKALEWLAHIFSTDEKSIRRSLRSRLTLSKDTSKSQVVLTMTNMDPVDTATYYCARDSSNYEGYFDYWGQGTLVTVSS

SEQ ID NO: 24 - protein, 107 aa, Artificial Sequence
  Synthetic Construct
EVVMTQSPATLSVSPGERATLSCRASQGVSSNFAWYQQRPGQSPRLLLYGASTRATGVPGRFSGSGSGTENILTISSLQSEDFAIYFCQQYKDWPFTFGPGSKVDIK

SEQ ID NO: 25 - protein, 121 aa, Artificial Sequence
  Synthetic Construct
QVTLEESGPVLVKPTETLTLTCTVSGFSLSNARMGVSWIRQPPGKAPEWFAHIFSTDEKSLRLSLRSRLTLSKDTSKSQVVLTMTNMDPVDTATYYCARDSSNYEGYFDYWGQGTLVTVSS

SEQ ID NO: 26 - protein, 107 aa, Artificial Sequence
  Synthetic Construct
EVVMTQSPATLSVSPGERATLSCRASQSVNRNLAWYQQKPGQAPRLLIFGTSTRATGIPARFSGSGSGTEFTLTIDSLQSEHSGLYYCQQYNDWPFTFGPGTKVDIK

SEQ ID NO: 27 - protein, 121 aa, Artificial Sequence
  Synthetic Construct
QVTLKESGPVLVKPTETLTLTCTVSGFSLSNAKMGVSWIRQPPGKALEWLAHIFSTDEKSIRRSLRSRLTMSKDTSKSQVVLTMTNMDPVDTATYYCVRDSSNYEGYFDYWGQGTLVTVSS

SEQ ID NO: 28 - protein, 107 aa, Artificial Sequence
  Synthetic Construct
EVLMTQSPATLSVSPGERATLSCRASQSVSTNFAWYQQRPGQAPRLLLFGASTRATGIPGRFSGSGSGTENILTISSLQSEDFAIYFCQQYKDWPFTFGPGSKVEIK

SEQ ID NO: 29 - protein, 107 aa, Artificial Sequence
  Synthetic Construct
DVVLTQSPATLSVSPGERATLSCRASQSVNSNLAWYQQNPGQAPRLLIFGSSTRATGIPASFSGSGSGTEFTLTINSLQSEHSAVYYCQQYNDWPFTFGPGTKVDIK

SEQ ID NO: 30 - protein, 121 aa, Artificial Sequence
  Synthetic Construct
QVTLKESGPVLVKPTETLTLTCTVSGFSLSNPRMGVSWIRQPPGKALEWLGHIFSSDEKSYRLSLRSRLSISKDTSKSQVVLTMTNMDPVDTATYYCVRDSSNYGGYFDYWGQGTLVTVSS

SEQ ID NO: 31 - protein, 107 aa, Artificial Sequence
  Synthetic Construct
EVVMTQSPATLSVSPGERATLSCRASQSVINNLAWYQQKPGQAPRLLIYGTSTRATDIPARFSGSGSGTEFTLTISSLQSEDFAVYYCQDYNNWPFTFGPGTKVDIK

SEQ ID NO: 32 - protein, 121 aa, Artificial Sequence
  Synthetic Construct
QVTLKESGPVLVKPIETLTLTCTVCGFSLSNPRMGVSWIRQPPGKALEWLGHIFSSDEKSYRLFLRSRLSISKDTSKSQVVLTMTNMDPVDTATYYCARDSSDYEGYFDYWGQGTLVTVSS

SEQ ID NO: 33 - protein, 107 aa, Artificial Sequence
  Synthetic Construct
EIVMTQSPATLSVSPGERTTLSCRASQSVGSNLAWYQQKPGQAPRLLIYGASTRASGVPARFSGSGSGTEFTLTISSLQSEDFAVYSCQEYNNWPFTFGQGTKVEIK

SEQ ID NO: 34 - protein, 121 aa, Artificial Sequence
  Synthetic Construct
  misc_feature (83)..(83): Xaa can be any naturally occurring amino acid
QVTLKESGPVLVKPTETLTLTCTVFGFSLSNPRMGVSWIRQPPGKAPEWLGHIFSSDEKSYRLSLRSRLSISKDTSKSQVVFXMTNMDPGDPATYYCVRDSSNYEEYFDYWGQGTLVTVSS

SEQ ID NO: 35 - protein, 121 aa, Artificial Sequence
  Synthetic Construct
QVTLKESGPVLVKPTETLTLTCTVSGFSLSNPRMGVSWLRQPPGKALEWFAHIFSTDEKSYSPSLRGRLTVSKDTSKSQVVLTLTNMDPVDTATYYCARDSSNYEGYFDYWGQGTLVTVSS

SEQ ID NO: 36 - protein, 107 aa, Artificial Sequence
  Synthetic Construct
KIVMTQSPATLSVSPGERATLSCRANQIVSSNLAWYQQKPGQAPRLLVFGTSTRATGIPIRFSGSGSGTEFTLTVSSLQSEDFAVYVCQQYNDWPFTFGPGTKVDIK

SEQ ID NO: 37 - protein, 118 aa, Artificial Sequence
  Synthetic Construct
EVQLVESGGGLVKPGGSLRLSCEASGFTFSDAWMSWVRQAPGKGLEWVGRIKSKTDGGTTDYVVPLNGRFIISRDDSRNTLYLQLNNLKTEDTAVYYCTTVPGSYGYWGQGTLVTVSS

SEQ ID NO: 38 - protein, 112 aa, Artificial Sequence
  Synthetic Construct
DIVMTQSPLSLPVTPGEPASISCRSSQSLLHNKRNNYLDWFLQKPGQSPQLLIYLASNRASGVPDRFSGGGSGTDFTLKISRVEAEDVGVYYCMQAQQTPITFGQGTRLEIK

SEQ ID NO: 39 - protein, 120 aa, Artificial Sequence
  Synthetic Construct
EVNLVESGGGLVKPGGSLRLSCEASGFTFSYAWMSWVRQAPGKGLEWVGRIKSIADGGATDYAAPVRNRFTISRDDSRNTLYLEMHSLKTEDTAVYYCTTIPGNDAFDMWGQGTMVTVSS

SEQ ID NO: 40 - protein, 112 aa, Artificial Sequence
  Synthetic Construct
DIVLTQSPLSLSVTPGEPASISCRSSQSLLYSNGKNYLDWFLHKPGQSPQLLIYLGSNRASGVPDRFSGSGSGIDFILKISRVEAEDVGVYYCMQAQQTPITFGQGTRLEIK

SEQ ID NO: 41 - protein, 119 aa, Artificial Sequence
  Synthetic Construct
EVQLVESWGVLVKPGGSLRLSCAASGFIFNNAWMSWVRQAPGKGLEWIGRIKSKSDGGTTDYAAPVKDRFTISRDDSKDTLYLQMNGLKTEDTAVYFCTTAPGGPFDYWGQGTLVTVSS

SEQ ID NO: 42 - protein, 112 aa, Artificial Sequence
  Synthetic Construct
DIVLTQSPLSLPVTPGEPASISCRSSQSLLHRDGFNYLDWFLQKPGQSPQLLIYLASSRASGVPDRFSGSDSGTDFTLKISRVEAEDVGVYYCMQALQTPITFGQGTRLEIK

SEQ ID NO: 43 - protein, 120 aa, Artificial Sequence
  Synthetic Construct
EVNLVESGGGLVKPGGSLRLSCEASGFTFSYAWMSWVRQAPGKGLEWVGRIKSITDGGVIDYAAPVRNRCTISRDDSRNTLYLEMHSLKTEDTAVYYCTTIPGNDDFDMWGQGRMVTVSS

SEQ ID NO: 44 - protein, 120 aa, Artificial Sequence
  Synthetic Construct
EVNLVESGGGLVKPGGSLRLSCEASGFTFSYAWMSWVRQAPGKGLEWVGRIKSINDGGATDYASPVRNRFTISRDDSRNMLYLEMHSLKTEDTAVYYCTTIPGNDAFDMWGQGTLVTVSS

SEQ ID NO: 45 - protein, 112 aa, Artificial Sequence
  Synthetic Construct
DIVLTQSPLSLSVTPGEPASISCRSTQSLLYSNGKNYLDWFLHKPGQSPQLLIFLGSIRASGVPDRFSGSGSGIDFILKISRVEAEDVGVYYCMQAQQTPITFGQGTRLEIK

SEQ ID NO: 46 - protein, 119 aa, Artificial Sequence
  Synthetic Construct
EVQLVESGGDLVKPGGSLRLSCAASGFTFTNAWMSWVRQAPGKGLEWVGRIKSKIDGGTTDYAAPVKGRFIISRDDSKNTLSLQMNSLKTEDTAMYYCTTAPGGPFDYWGQGSLVTVSS

SEQ ID NO: 47 - protein, 112 aa, Artificial Sequence
  Synthetic Construct
DIVLTQSPLSLPVTPGEPASISCRSSQSLLYSDRRNYLDWFLQKPGQSPHLLIYLGSYRASGVPDRFSGSGSGTDFTLKISRVEAEDVGVYYCMQALQIPITFGQGTRLEIK

SEQ ID NO: 48 - protein, 126 aa, Artificial Sequence
  Synthetic Construct
QVQLVQSGAEVKKPGSSVKVSCKASGDTFSSNAISWVRQAPGQGLEWMGVIIPIFGTADYAQKFQGRVTITADESTSTAYMELSSLRSEDTAVYYCARHTYHEYAGGYYGGAMDPWGQGTLVTVSS

SEQ ID NO: 49 - protein, 112 aa, Artificial Sequence
  Synthetic Construct
ELQSVLTQPPSASGTPGQRVTISCSGSSSNIGSNYVYWYQQLPGTAPKILIYRNNQRPSGVPDRFSGSKSGTSASLAISGLRSEDEADYYCAAWDDNLSGWVFGTGTKLTVL

SEQ ID NO: 50 - protein, 123 aa, Artificial Sequence
  Synthetic Construct
EVQLLESGGGLVQPGGSLRLSCAASGFTFSNYAMSWVRQAPGKGLEWVSDISGGGGRTYYADSVKGRFTISRDNSKNTLYLQMNSLRAEDTAVYYCARAGLLYGGGVYPMDIWGQGTLVTVSS

SEQ ID NO: 51 - protein, 107 aa, Artificial Sequence [sequence omitted]

SEQ ID NO: 52 - protein, 491 aa, Artificial Sequence
  Synthetic Construct
MALPVTALLLPLALLLHAARPDVVMTQSPLSLPVTLGQPASISCKSSQSLLYSNGKTYLNWFQQRPGQSPRRLIYQVSKLDSGVPDRFSGSGSGTDFTLKISRVEAEDVGVYYCGQDTHFPLTFGGGTKVEIKGGGGSGGGGSGGGGSGGGGSQVQLVQSGAEVKKPGASVKVSCKASGYTFTDYTLHWVRQAPGQGLEWMGGIWPITGGTTYNQKFKGRVTMTRDTSTSTVYMELSSLRSEDTAVYYCARGEAQGSWGQGTLVTVSSTTTPAPRPPTPAPTIASQPLSLRPEACRPAAGGAVHTRGLDFACDIYIWAPLAGTCGVLLLSLVITLYCKRGRKKLLYIFKQPFMRPVQTTQEEDGCSCRFPEEEEGGCELRVKFSRSADAPAYQQGQNQLYNELNLGRREEYDVLDKRRGRDPEMGGKPRRKNPQEGLYNELQKDKMAEAYSEIGMKGERRRGKGHDGLYQGLSTATKDTYDALHMQALPPR

SEQ ID NO: 53 - protein, 492 aa, Artificial Sequence
  Synthetic Construct
MALPVTALLLPLALLLHAARPQVTLKESGPVLLKPTETLTLTCTVSGFSLSNPRMGVSWIRQPPGKALEWFAHIFSTDEKSLKLSLRSRLTLSKDTSKSQVVLTMTNMAPVDSATYYCARDSSNYEGYFDFWGQGTLVTVSSGGGGSGGGGSGGGGSGGGGSEVVLTQSPATLSVSPGERATLSCRASQSVRSNLAWYQQKSGQAPRLLIYGSTIRATGVPARFSGSGSGTEFTLTISSLQSEDFAVYYCQQYSDWPFTFGPGTKVDIKTTTPAPRPPTPAPTIASQPLSLRPEACRPAAGGAVHTRGLDFACDIYIWAPLAGTCGVLLLSLVITLYCKRGRKKLLYIFKQPFMRPVQTTQEEDGCSCRFPEEEEGGCELRVKFSRSADAPAYQQGQNQLYNELNLGRREEYDVLDKRRGRDPEMGGKPRRKNPQEGLYNELQKDKMAEAYSEIGMKGERRRGKGHDGLYQGLSTATKDTYDALHMQALPPR

SEQ ID NO: 54 - protein, 492 aa, Artificial Sequence
  Synthetic Construct
MALPVTALLLPLALLLHAARPQVTLKESGPVLVKPTETLTLTCTVSGFSLSNARMGVSWIRQPPGKALEWLAHIFSTDEKSIRRSLRSRLTLSKDTSKSQVVLTMTNMDPVDTATYFCARDSSNYEGYFDYWGQGTLVTVSSGGGGSGGGGSGGGGSGGGGSEVVMTQSPATLSVSPGERVTLSCRASQSVSSNFAWYQQRPGQAPRLLLYGATTRATGLPGRFSGSGSGTENILTISSLQSEDFAIYFCQQYKDWPFTFGPGSKVDIKTTTPAPRPPTPAPTIASQPLSLRPEACRPAAGGAVHTRGLDFACDIYIWAPLAGTCGVLLLSLVITLYCKRGRKKLLYIFKQPFMRPVQTTQEEDGCSCRFPEEEEGGCELRVKFSRSADAPAYQQGQNQLYNELNLGRREEYDVLDKRRGRDPEMGGKPRRKNPQEGLYNELQKDKMAEAYSEIGMKGERRRGKGHDGLYQGLSTATKDTYDALHMQALPPR

SEQ ID NO: 55 - protein, 492 aa, Artificial Sequence
  Synthetic Construct
MALPVTALLLPLALLLHAARPQVTLKESGPVLVKPTETLTLTCTVSGFSLSNARMGVSWIRQPPGKALEWLGHIFSTDEKSYSTSLRGRITISKDTSRGLVVLTLTNMDPVDTATYYCARDSSNYEGYFDFWGPGFLVTVSSGGGGSGGGGSGGGGSGGGGSEIVMTQSPATLSVSPGERATLSCRVSQSIGANLAWYQQKFGQAPRLLIYGASTRATGIPVRFSGGGSGTEFTLTISSLQSEDFAIYSCQQYIYWPFTFGPGTTVDIKTTTPAPRPPTPAPTIASQPLSLRPEACRPAAGGAVHTRGLDFACDIYIWAPLAGTCGVLLLSLVITLYCKRGRKKLLYIFKQPFMRPVQTTQEEDGCSCRFPEEEEGGCELRVKFSRSADAPAYQQGQNQLYNELNLGRREEYDVLDKRRGRDPEMGGKPRRKNPQEGLYNELQKDKMAEAYSEIGMKGERRRGKGHDGLYQGLSTATKDTYDALHMQALPPR

SEQ ID NO: 56 - protein, 492 aa, Artificial Sequence
  Synthetic Construct
MALPVTALLLPLALLLHAARPQVTLKESGPVLVKPTETLTLTCTVSGFSLNNARMGVSWIRQPPGKALEWFAHIFSTDEKSFRTSLRSRLTLSKDTSKSQVVLTMTNMDPVDTATYYCARDSSNYEGYFDYWGQGILVTVSSGGGGSGGGGSGGGGSGGGGSEIVMTQSPATLSVSPGERATLSCRASQSVSNNLAWYQQKPGQAPRLLIYGASTRATGVPARFSGSDSGTEFSLTISSLQSEDFAVYFCQQYKDWPFTFGPGTKVEIKTTTPAPRPPTPAPTIASQPLSLRPEACRPAAGGAVHTRGLDFACDIYIWAPLAGTCGVLLLSLVITLYCKRGRKKLLYIFKQPFMRPVQTTQEEDGCSCRFPEEEEGGCELRVKFSRSADAPAYQQGQNQLYNELNLGRREEYDVLDKRRGRDPEMGGKPRRKNPQEGLYNELQKDKMAEAYSEIGMKGERRRGKGHDGLYQGLSTATKDTYDALHMQALPPR

SEQ ID NO: 57 - protein, 496 aa, Artificial Sequence
  Synthetic Construct
MALPVTALLLPLALLLHAARPEVNLVESGGGLVKPGGSLRLSCEASGFTFSYAWMSWVRQAPGKGLEWVGRIKSIADGGATDYAAPVRNRFTISRDDSRNTLYLEMHSLKTEDTAVYYCTTIPGNDAFDMWGQGTMVTVSSGGGGSGGGGSGGGGSGGGGSDIVLTQSPLSLSVTPGEPASISCRSSQSLLYSNGKNYLDWFLHKPGQSPQLLIYLGSNRASGVPDRFSGSGSGIDFILKISRVEAEDVGVYYCMQAQQTPITFGQGTRLEIKTTTPAPRPPTPAPTIASQPLSLRPEACRPAAGGAVHTRGLDFACDIYIWAPLAGTCGVLLLSLVITLYCKRGRKKLLYIFKQPFMRPVQTTQEEDGCSCRFPEEEEGGCELRVKFSRSADAPAYQQGQNQLYNELNLGRREEYDVLDKRRGRDPEMGGKPRRKNPQEGLYNELQKDKMAEAYSEIGMKGERRRGKGHDGLYQGLSTATKDTYDALHMQALPPR

SEQ ID NO: 58 - protein, 496 aa, Artificial Sequence
  Synthetic Construct
MALPVTALLLPLALLLHAARPEVNLVESGGGLVKPGGSLRLSCEASGFTFSYAWMSWVRQAPGKGLEWVGRIKSITDGGVIDYAAPVRNRCTISRDDSRNTLYLEMHSLKTEDTAVYYCTTIPGNDDFDMWGQGRMVTVSSGGGGSGGGGSGGGGSGGGGSDIVLTQSPLSLSVTPGEPASISCRSSQSLLYSNGKNYLDWFLHKPGQSPQLLIYLGSNRASGVPDRFSGSGSGIDFILKISRVEAEDVGVYYCMQAQQTPITFGQGTRLEIKTTTPAPRPPTPAPTIASQPLSLRPEACRPAAGGAVHTRGLDFACDIYIWAPLAGTCGVLLLSLVITLYCKRGRKKLLYIFKQPFMRPVQTTQEEDGCSCRFPEEEEGGCELRVKFSRSADAPAYQQGQNQLYNELNLGRREEYDVLDKRRGRDPEMGGKPRRKNPQEGLYNELQKDKMAEAYSEIGMKGERRRGKGHDGLYQGLSTATKDTYDALHMQALPPR

SEQ ID NO: 59 - protein, 495 aa, Artificial Sequence
  Synthetic Construct
MALPVTALLLPLALLLHAARPEVQLVESWGVLVKPGGSLRLSCAASGFIFNNAWMSWVRQAPGKGLEWIGRIKSKSDGGTTDYAAPVKDRFTISRDDSKDTLYLQMNGLKTEDTAVYFCTTAPGGPFDYWGQGTLVTVSSGGGGSGGGGSGGGGSGGGGSDIVLTQSPLSLPVTPGEPASISCRSSQSLLHRDGFNYLDWFLQKPGQSPQLLIYLASSRASGVPDRFSGSDSGTDFTLKISRVEAEDVGVYYCMQALQTPITFGQGTRLEIKTTTPAPRPPTPAPTIASQPLSLRPEACRPAAGGAVHTRGLDFACDIYIWAPLAGTCGVLLLSLVITLYCKRGRKKLLYIFKQPFMRPVQTTQEEDGCSCRFPEEEEGGCELRVKFSRSADAPAYQQGQNQLYNELNLGRREEYDVLDKRRGRDPEMGGKPRRKNPQEGLYNELQKDKMAEAYSEIGMKGERRRGKGHDGLYQGLSTATKDTYDALHMQALPPR

SEQ ID NO: 60 - protein, 494 aa, Artificial Sequence
  Synthetic Construct
MALPVTALLLPLALLLHAARPEVQLVESGGGLVKPGGSLRLSCEASGFTFSDAWMSWVRQAPGKGLEWVGRIKSKTDGGTTDYVVPLNGRFIISRDDSRNTLYLQLNNLKTEDTAVYYCTTVPGSYGYWGQGTLVTVSSGGGGSGGGGSGGGGSGGGGSDIVMTQSPLSLPVTPGEPASISCRSSQSLLHNKRNNYLDWFLQKPGQSPQLLIYLASNRASGVPDRFSGGGSGTDFTLKISRVEAEDVGVYYCMQAQQTPITFGQGTRLEIKTTTPAPRPPTPAPTIASQPLSLRPEACRPAAGGAVHTRGLDFACDIYIWAPLAGTCGVLLLSLVITLYCKRGRKKLLYIFKQPFMRPVQTTQEEDGCSCRFPEEEEGGCELRVKFSRSADAPAYQQGQNQLYNELNLGRREEYDVLDKRRGRDPEMGGKPRRKNPQEGLYNELQKDKMAEAYSEIGMKGERRRGKGHDGLYQGLSTATKDTYDALHMQALPPR

SEQ ID NO: 61 - protein, 502 aa, Artificial Sequence
  Synthetic Construct
MALPVTALLLPLALLLHAARPQVQLVQSGAEVKKPGSSVKVSCKASGDTFSSNAISWVRQAPGQGLEWMGVIIPIFGTADYAQKFQGRVTITADESTSTAYMELSSLRSEDTAVYYCARHTYHEYAGGYYGGAMDPWGQGTLVTVSSGGGGSGGGGSGGGGSGGGGSELQSVLTQPPSASGTPGQRVTISCSGSSSNIGSNYVYWYQQLPGTAPKILIYRNNQRPSGVPDRFSGSKSGTSASLAISGLRSEDEADYYCAAWDDNLSGWVFGTGTKLTVLTTTPAPRPPTPAPTIASQPLSLRPEACRPAAGGAVHTRGLDFACDIYIWAPLAGTCGVLLLSLVITLYCKRGRKKLLYIFKQPFMRPVQTTQEEDGCSCRFPEEEEGGCELRVKFSRSADAPAYQQGQNQLYNELNLGRREEYDVLDKRRGRDPEMGGKPRRKNPQEGLYNELQKDKMAEAYSEIGMKGERRRGKGHDGLYQGLSTATKDTYDALHMQALPPR

SEQ ID NO: 62 - protein, 6 aa, Artificial Sequence
  Synthetic Construct
TDYTLH

SEQ ID NO: 63 - protein, 6 aa, Artificial Sequence
  Synthetic Construct
GYTFTD

SEQ ID NO: 64 - protein, 10 aa, Artificial Sequence
  Synthetic Construct
GYTFTDYTLH

SEQ ID NO: 65 - protein, 17 aa, Artificial Sequence
  Synthetic Construct
GIDPINGGTTYNQKFKG

SEQ ID NO: 66 - protein, 11 aa, Artificial Sequence
  Synthetic Construct
GIDPINGGTTY

SEQ ID NO: 67 - protein, 6 aa, Artificial Sequence
  Synthetic Construct
GEAMDS

SEQ ID NO: 68 - protein, 17 aa, Artificial Sequence
  Synthetic Construct
GINPINGGTTYNQKFKG

SEQ ID NO: 69 - protein, 11 aa, Artificial Sequence
  Synthetic Construct
GINPINGGTTY

SEQ ID NO: 70 - protein, 17 aa, Artificial Sequence
  Synthetic Construct
GIWPITGGTTYNQKFKG

SEQ ID NO: 71 - protein, 11 aa, Artificial Sequence
  Synthetic Construct
GIWPITGGTTY

SEQ ID NO: 72 - protein, 6 aa, Artificial Sequence
  Synthetic Construct
GEAEGS

SEQ ID NO: 73 - protein, 6 aa, Artificial Sequence
  Synthetic Construct
GEAQGS

SEQ ID NO: 74 - protein, 8 aa, Artificial Sequence
  Synthetic Construct
SNPRMGVS

SEQ ID NO: 75 - protein, 8 aa, Artificial Sequence
  Synthetic Construct
GFSLSNPR

SEQ ID NO: 76 - protein, 12 aa, Artificial Sequence
  Synthetic Construct
GFSLSNPRMGVS

SEQ ID NO: 77 - protein, 16 aa, Artificial Sequence
  Synthetic Construct
HIFSTDEKSLKLSLRS

SEQ ID NO: 78 - protein, 10 aa, Artificial Sequence
  Synthetic Construct
HIFSTDEKSL

SEQ ID NO: 79 - protein, 11 aa, Artificial Sequence
  Synthetic Construct
DSSNYEGYFDF

SEQ ID NO: 80 - protein, 8 aa, Artificial Sequence
  Synthetic Construct
SNARMGVS

SEQ ID NO: 81 - protein, 8 aa, Artificial Sequence
  Synthetic Construct
GFSLSNAR

SEQ ID NO: 82 - protein, 12 aa, Artificial Sequence
  Synthetic Construct
GFSLSNARMGVS

SEQ ID NO: 83 - protein, 16 aa, Artificial Sequence
  Synthetic Construct
HIFSTDEKSIRRSLRS

SEQ ID NO: 84 - protein, 10 aa, Artificial Sequence
  Synthetic Construct
HIFSTDEKSI

SEQ ID NO: 85 - protein, 11 aa, Artificial Sequence
  Synthetic Construct
DSSNYEGYFDY

SEQ ID NO: 86 - protein, 16 aa, Artificial Sequence
  Synthetic Construct
HIFSTDEKSYSTSLRG

SEQ ID NO: 87 - protein, 10 aa, Artificial Sequence
  Synthetic Construct
HIFSTDEKSY

SEQ ID NO: 88 - protein, 8 aa, Artificial Sequence
  Synthetic Construct
NNARMGVS

SEQ ID NO: 89 - protein, 8 aa, Artificial Sequence
  Synthetic Construct
GFSLNNAR

SEQ ID NO: 90 - protein, 12 aa, Artificial Sequence
  Synthetic Construct
GFSLNNARMGVS

SEQ ID NO: 91 - protein, 16 aa, Artificial Sequence
  Synthetic Construct
HIFSTDEKSFRTSLRS

SEQ ID NO: 92 - protein, 10 aa, Artificial Sequence
  Synthetic Construct
HIFSTDEKSF

SEQ ID NO: 93 - protein, 8 aa, Artificial Sequence
  Synthetic Construct
SNVRMGVS

SEQ ID NO: 94 - protein, 8 aa, Artificial Sequence
  Synthetic Construct
GFSLSNVR

SEQ ID NO: 95 - protein, 12 aa, Artificial Sequence
  Synthetic Construct
GFSLSNVRMGVS

SEQ ID NO: 96 - protein, 16 aa, Artificial Sequence
  Synthetic Construct
HIFSSDEKSIRRSLRS

SEQ ID NO: 97 - protein, 10 aa, Artificial Sequence
  Synthetic Construct
HIFSSDEKSI

SEQ ID NO: 98 - protein, 16 aa, Artificial Sequence
  Synthetic Construct
HIFSTDEKSLRLSLRS

SEQ ID NO: 99 - protein, 8 aa, Artificial Sequence
  Synthetic Construct
SNAKMGVS

SEQ ID NO: 100 - protein, 8 aa, Artificial Sequence
  Synthetic Construct
GFSLSNAK

SEQ ID NO: 101 - protein, 12 aa, Artificial Sequence
  Synthetic Construct
GFSLSNAKMGVS

SEQ ID NO: 102 - protein, 16 aa, Artificial Sequence
  Synthetic Construct
HIFSSDEKSYRLSLRS

SEQ ID NO: 103 - protein, 10 aa, Artificial Sequence
  Synthetic Construct
HIFSSDEKSY

SEQ ID NO: 104 - protein, 11 aa, Artificial Sequence
  Synthetic Construct
DSSNYGGYFDY

SEQ ID NO: 105 - protein, 16 aa, Artificial Sequence
  Synthetic Construct
HIFSSDEKSYRLFLRS

SEQ ID NO: 106 - protein, 16 aa, Artificial Sequence
  Synthetic Construct
HIFSTDEKSYSPSLRG

SEQ ID NO: 107 - protein, 11 aa, Artificial Sequence
  Synthetic Construct
DSSDYEGYFDY

SEQ ID NO: 108 - protein, 11 aa, Artificial Sequence
  Synthetic Construct
DSSNYEEYFDY

SEQ ID NO: 109 - protein, 6 aa, Artificial Sequence
  Synthetic Construct
SDAWMS

SEQ ID NO: 110 - protein, 6 aa, Artificial Sequence
  Synthetic Construct
GFTFSD

SEQ ID NO: 111 - protein, 10 aa, Artificial Sequence
  Synthetic Construct
GFTFSDAWMS

SEQ ID NO: 112 - protein, 19 aa, Artificial Sequence
  Synthetic Construct
RIKSKTDGGTTDYVVPLNG

SEQ ID NO: 113 - protein, 13 aa, Artificial Sequence
  Synthetic Construct
RIKSKTDGGTTDY

SEQ ID NO: 114 - protein, 7 aa, Artificial Sequence
  Synthetic Construct
VPGSYGY

SEQ ID NO: 115 - protein, 6 aa, Artificial Sequence
  Synthetic Construct
SYAWMS

SEQ ID NO: 116 - protein, 6 aa, Artificial Sequence
  Synthetic Construct
GFTFSY

SEQ ID NO: 117 - protein, 10 aa, Artificial Sequence
  Synthetic Construct
GFTFSYAWMS

SEQ ID NO: 118 - protein, 19 aa, Artificial Sequence
  Synthetic Construct
RIKSIADGGATDYAAPVRN

SEQ ID NO: 119 - protein, 13 aa, Artificial Sequence
  Synthetic Construct
RIKSIADGGATDY

SEQ ID NO: 120 - protein, 9 aa, Artificial Sequence
  Synthetic Construct
IPGNDAFDM

SEQ ID NO: 121 - protein, 6 aa, Artificial Sequence
  Synthetic Construct
NNAWMS

SEQ ID NO: 122 - protein, 6 aa, Artificial Sequence
  Synthetic Construct
GFIFNN

SEQ ID NO: 123 - protein, 10 aa, Artificial Sequence
  Synthetic Construct
GFIFNNAWMS

SEQ ID NO: 124 - protein, 19 aa, Artificial Sequence
  Synthetic Construct
RIKSKSDGGTTDYAAPVKD

SEQ ID NO: 125 - protein, 13 aa, Artificial Sequence
  Synthetic Construct
RIKSKSDGGTTDY

SEQ ID NO: 126 - protein, 8 aa, Artificial Sequence
  Synthetic Construct
APGGPFDY

SEQ ID NO: 127 - protein, 19 aa, Artificial Sequence
  Synthetic Construct
RIKSITDGGVIDYAAPVRN

SEQ ID NO: 128 - protein, 13 aa, Artificial Sequence
  Synthetic Construct
RIKSITDGGVIDY

SEQ ID NO: 129 - protein, 9 aa, Artificial Sequence
  Synthetic Construct
IPGNDDFDM

SEQ ID NO: 130 - protein, 19 aa, Artificial Sequence
  Synthetic Construct
RIKSINDGGATDYASPVRN

SEQ ID NO: 131 - protein, 13 aa, Artificial Sequence
  Synthetic Construct
RIKSINDGGATDY

SEQ ID NO: 132 - protein, 6 aa, Artificial Sequence
  Synthetic Construct
TNAWMS

SEQ ID NO: 133 - protein, 6 aa, Artificial Sequence
  Synthetic Construct
GFTFTN

SEQ ID NO: 134 - protein, 10 aa, Artificial Sequence
  Synthetic Construct
GFTFTNAWMS

SEQ ID NO: 135 - protein, 19 aa, Artificial Sequence
  Synthetic Construct
RIKSKIDGGTTDYAAPVKG

SEQ ID NO: 136 - protein, 13 aa, Artificial Sequence
  Synthetic Construct
RIKSKIDGGTTDY

SEQ ID NO: 137 - protein, 6 aa, Artificial Sequence
  Synthetic Construct
SSNAIS

SEQ ID NO: 138 - protein, 6 aa, Artificial Sequence
  Synthetic Construct
GDTFSS

SEQ ID NO: 139 - protein, 10 aa, Artificial Sequence
  Synthetic Construct
GDTFSSNAIS

SEQ ID NO: 140 - protein, 17 aa, Artificial Sequence
  Synthetic Construct
VIIPIFGTADYAQKFQG

SEQ ID NO: 141 - protein, 11 aa, Artificial Sequence
  Synthetic Construct
VIIPIFGTADY

SEQ ID NO: 142 - protein, 17 aa, Artificial Sequence
  Synthetic Construct
HTYHEYAGGYYGGAMDP

SEQ ID NO: 143 - protein, 6 aa, Artificial Sequence
  Synthetic Construct
SNYAMS

SEQ ID NO: 144 - protein, 6 aa, Artificial Sequence
  Synthetic Construct
GFTFSN

SEQ ID NO: 145 - protein, 10 aa, Artificial Sequence
  Synthetic Construct
GFTFSNYAMS

SEQ ID NO: 146 - protein, 17 aa, Artificial Sequence
  Synthetic Construct
DISGGGGRTYYADSVKG

SEQ ID NO: 147 - protein, 11 aa, Artificial Sequence
  Synthetic Construct
DISGGGGRTYY

SEQ ID NO: 148 - protein, 14 aa, Artificial Sequence
  Synthetic Construct
AGLLYGGGVYPMDI

SEQ ID NO: 149 - protein, 16 aa, Artificial Sequence
  Synthetic Construct
KSSQSLLYSNGKTYLN

SEQ ID NO: 150 - protein, 7 aa, Artificial Sequence
  Synthetic Construct
LVSKLDS

SEQ ID NO: 151 - protein, 9 aa, Artificial Sequence
  Synthetic Construct
VQDTHFPLT

SEQ ID NO: 152 - protein, 7 aa, Artificial Sequence
  Synthetic Construct
QVSKLDS

SEQ ID NO: 153 - protein, 9 aa, Artificial Sequence
  Synthetic Construct
GQDTHFPLT

SEQ ID NO: 154 - protein, 16 aa, Artificial Sequence
  Synthetic Construct
KSSQSLLYSNDKTYTN

SEQ ID NO: 155 - protein, 7 aa, Artificial Sequence
  Synthetic Construct
EVSKLDV

SEQ ID NO: 156 - protein, 11 aa, Artificial Sequence
  Synthetic Construct
RASQSVRSNLA

SEQ ID NO: 157 - protein, 7 aa, Artificial Sequence
  Synthetic Construct
GSTIRAT

SEQ ID NO: 158 - protein, 9 aa, Artificial Sequence
  Synthetic Construct
QQYSDWPFT

SEQ ID NO: 159 - protein, 11 aa, Artificial Sequence
  Synthetic Construct
RASQSVSSNFA

SEQ ID NO: 160 - protein, 7 aa, Artificial Sequence
  Synthetic Construct
GATTRAT

SEQ ID NO: 161 - protein, 9 aa, Artificial Sequence
  Synthetic Construct
QQYKDWPFT

SEQ ID NO: 162 - protein, 11 aa, Artificial Sequence
  Synthetic Construct
RVSQSIGANLA

SEQ ID NO: 163 - protein, 7 aa, Artificial Sequence
  Synthetic Construct
GASTRAT

SEQ ID NO: 164 - protein, 9 aa, Artificial Sequence
  Synthetic Construct
QQYIYWPFT

SEQ ID NO: 165 - protein, 11 aa, Artificial Sequence
  Synthetic Construct
RASQSVSNNLA

SEQ ID NO: 166 - protein, 11 aa, Artificial Sequence
  Synthetic Construct
RASQSVGSDLA

SEQ ID NO: 167 - protein, 9 aa, Artificial Sequence
  Synthetic Construct
QQYNDWPFT

SEQ ID NO: 168 - protein, 11 aa, Artificial Sequence
  Synthetic Construct
RASQNIGSDLA

SEQ ID NO: 169 - protein, 11 aa, Artificial Sequence
  Synthetic Construct
RASQSVTSNFA

SEQ ID NO: 170 - protein, 11 aa, Artificial Sequence
  Synthetic Construct
RASQGVSSNFA

SEQ ID NO: 171 - protein, 11 aa, Artificial Sequence
  Synthetic Construct
RASQSVNRNLA

SEQ ID NO: 172 - protein, 7 aa, Artificial Sequence
  Synthetic Construct
GTSTRAT

SEQ ID NO: 173 - protein, 11 aa, Artificial Sequence
  Synthetic Construct
RASQSVSTNFA

SEQ ID NO: 174 - protein, 11 aa, Artificial Sequence
  Synthetic Construct
RASQSVNSNLA

SEQ ID NO: 175 - protein, 7 aa, Artificial Sequence
  Synthetic Construct
GSSTRAT

SEQ ID NO: 176 - protein, 11 aa, Artificial Sequence
  Synthetic Construct
RASQSVINNLA

SEQ ID NO: 177 - protein, 9 aa, Artificial Sequence
  Synthetic Construct
QDYNNWPFT

SEQ ID NO: 178 - protein, 11 aa, Artificial Sequence
  Synthetic Construct
RASQSVGSNLA

SEQ ID NO: 179 - protein, 8 aa, Artificial Sequence
  Synthetic Construct
GASTRASG

SEQ ID NO: 180 - protein, 9 aa, Artificial Sequence
  Synthetic Construct
QEYNNWPFT

SEQ ID NO: 181 - protein, 11 aa, Artificial Sequence
  Synthetic Construct
RANQIVSSNLA

SEQ ID NO: 182 - protein, 16 aa, Artificial Sequence
  Synthetic Construct
RSSQSLLHNKRNNYLD

SEQ ID NO: 183 - protein, 7 aa, Artificial Sequence
  Synthetic Construct
LASNRAS

SEQ ID NO: 184 - protein, 9 aa, Artificial Sequence
  Synthetic Construct
MQAQQTPIT

SEQ ID NO: 185 - protein, 16 aa, Artificial Sequence
  Synthetic Construct
RSSQSLLYSNGKNYLD

SEQ ID NO: 186 - protein, 7 aa, Artificial Sequence
  Synthetic Construct
LGSNRAS

SEQ ID NO: 187 - protein, 16 aa, Artificial Sequence
  Synthetic Construct
RSSQSLLHRDGFNYLD

SEQ ID NO: 188 - protein, 7 aa, Artificial Sequence
  Synthetic Construct
LASSRAS

SEQ ID NO: 189 - protein, 9 aa, Artificial Sequence
  Synthetic Construct
MQALQTPIT

SEQ ID NO: 190 - protein, 16 aa, Artificial Sequence
  Synthetic Construct
RSTQSLLYSNGKNYLD

SEQ ID NO: 191 - protein, 7 aa, Artificial Sequence
  Synthetic Construct
LGSIRAS

SEQ ID NO: 192 - protein, 16 aa, Artificial Sequence
  Synthetic Construct
RSSQSLLYSDRRNYLD

SEQ ID NO: 193 - protein, 7 aa, Artificial Sequence
  Synthetic Construct
LGSYRAS

SEQ ID NO: 194 - protein, 9 aa, Artificial Sequence
  Synthetic Construct
MQALQIPIT

SEQ ID NO: 195 - protein, 13 aa, Artificial Sequence
  Synthetic Construct
SGSSSNIGSNYVY

SEQ ID NO: 196 - protein, 7 aa, Artificial Sequence
  Synthetic Construct
RNNQRPS

SEQ ID NO: 197 - protein, 11 aa, Artificial Sequence
  Synthetic Construct
AAWDDNLSGWV

SEQ ID NO: 198 - protein, 11 aa, Artificial Sequence
  Synthetic Construct
RASQSISSYLN

SEQ ID NO: 199 - protein, 7 aa, Artificial Sequence
  Synthetic Construct
AASSLQS

SEQ ID NO: 200 - protein, 9 aa, Artificial Sequence
  Synthetic Construct
QQSYSTPLT

SEQ ID NO: 201 - protein, 943 aa, Homo sapien
MRPSGTAGAALLALLAALCPASRALEEKKGNYVVTDHGSCVRACGADSYEMEEDGVRKCKKCEGPCRKVCNGIGIGEFKDSLSINATNIKHFKNCTSISGDLHILPVAFRGDSFTHTPPLDPQELDILKTVKEITGFLLIQAWPENRTDLHAFENLEIIRGRTKQHGQFSLAVVSLNITSLGLRSLKEISDGDVIISGNKNLCYANTINWKKLFGTSGQKTKIISNRGENSCKATGQVCHALCSPEGCWGPEPRDCVSCRNVSRGRECVDKCNLLEGEPREFVENSECIQCHPECLPQAMNITCTGRGPDNCIQCAHYIDGPHCVKTCPAGVMGENNTLVWKYADAGHVCHLCHPNCTYGCTGPGLEGCPTNGPKIPSIATGMVGALLLLLVVALGIGLFMRRRHIVRKRTLRRLLQERELVEPLTPSGEAPNQALLRILKETEFKKIKVLGSGAFGTVYKGLWIPEGEKVKIPVAIKELREATSPKANKEILDEAYVMASVDNPHVCRLLGICLTSTVQLITQLMPFGCLLDYVREHKDNIGSQYLLNWCVQIAKGMNYLEDRRLVHRDLAARNVLVKTPQHVKITDFGLAKLLGAEEKEYHAEGGKVPIKWMALESILHRIYTHQSDVWSYGVTVWELMTFGSKPYDGIPASEISSILEKGERLPQPPICTIDVYMIMVKCWMIDADSRPKFRELIIEFSKMARDPQRYLVIQGDERMHLPSPTDSNFYRALMDEEDMDDVVDADEYLIPQQGFFSSPSTSRTPLLSSLSATSNNSTVACIDRNGLQSCPIKEDSFLQRYSSDPTGALTEDSIDDTFLPVPEYINQSVPKRPAGSVQNPVYHNQPLNPAPSRDPHYQDPHSTAVGNPEYLNTVQPTCVNSTFDSPAHWAQKGSHQISLDNPDYQQDFFPKEAKPNGIFKGSTAENAEYLRVAPQSSEFIGA

SEQ ID NO: 202 - protein, 20 aa, Artificial Sequence
  Synthetic Construct
GGGGSGGGGSGGGGSGGGGS

SEQ ID NO: 203 - protein, 42 aa, Homo sapien
KRGRKKLLYIFKQPFMRPVQTTQEEDGCSCRFPEEEEGGCEL

SEQ ID NO: 204 - protein, 42 aa, Homo sapien; identical to SEQ ID NO: 203

SEQ ID NO: 205 - protein, 112 aa, Homo sapien
RVKFSRSADAPAYQQGQNQLYNELNLGRREEYDVLDKRRGRDPEMGGKPRRKNPQEGLYNELQKDKMAEAYSEIGMKGERRRGKGHDGLYQGLSTATKDTYDALHMQALPPR

SEQ ID NO: 206 - protein, 21 aa, Homo sapien
MALPVTALLLPLALLLHAARP

SEQ ID NO: 207 - protein, 16 aa, Homo sapien
GLAVSTISSFFPPGYQ

SEQ ID NO: 208 - protein, 45 aa, Homo sapien
TTTPAPRPPTPAPTIASQPLSLRPEACRPAAGGAVHTRGLDFACD

SEQ ID NO: 209 - protein, 231 aa, Homo sapien
EPKSPDKTHTCPPCPAPPVAGPSVFLFPPKPKDTLMIARTPEVTCVVVDVSHEDPEVKFNWYVDGVEVHNAKTKPREEQYNSTYRVVSVLTVLHQDWLNGKEYKCKVSNKALPAPIEKTISKAKGQPREPQVYTLPPSRDELTKNQVSLTCLVKGFYPSDIAVEWESNGQPENNYKTTPPVLDSDGSFFLYSKLTVDKSRWQQGNVFSCSVMHEALHNHYTQKSLSLSPGK

SEQ ID NO: 210 - protein, 24 aa, Homo sapien
IYIWAPLAGTCGVLLLSLVITLYC

SEQ ID NO: 211 - protein, 52 aa, Homo sapien
FFIPLLVVILFAVDTGLFISTQQQVTFLLKIKRTRKGFRLLNPHPKPNPKNN

SEQ ID NO: 212 - protein, 215 aa, Homo sapien
MDTESNRRANLALPQEPSSVPAFEVLEISPQEVSSGRLLKSASSPPLHTWLTVLKKEQEFLGVTQILTAMICLCFGTVVCSVLDISHIEGDIFSSFKAGYPFWGAIFFSISGMLSIISERRNATYLVRGSLGANTASSIAGGTGITILIINLKKSLAYIHIHSCQKFFETKCFMASFSTEIVVMMLFLTILGLGSAVSLTICGAGEELKGNKVPE

SEQ ID NO: 213 - protein, 41 aa, Homo sapien
RSKRSRGGHSDYMNMTPRRPGPTRKHYQPYAPPRDFAAYRS

SEQ ID NO: 214 - protein, 18 aa, Homo sapien
MIPAVVLLLLLLVEQAAA

SEQ ID NO: 215 - protein, 43 aa, Artificial Sequence
  Synthetic Construct
LGEPQLCYILDAILFLYGIVLTLLYCRLKIQVRKAAITSYEKS

SEQ ID NO: 216 - protein, 22 aa, Homo sapien
GSGATNFSLLKQAGDVEENPGP

SEQ ID NO: 217 - protein, 21 aa, Homo sapien
GSGEGRGSLLTCGDVEENPGP

SEQ ID NO: 218 - protein, 530 aa, Homo sapien
LTPQQVVAIASNGGGKQALETVQRLLPVLCQAHGLTPQQVVAIASNNGGKQALETVQRLLPVLCQAHGLTPQQVVAIASNGGGKQALETVQRLLPVLCQAHGLTPEQVVAIASHDGGKQALETVQRLLPVLCQAHGLTPEQVVAIASHDGGKQALETVQRLLPVLCQAHGLTPEQVVAIASHDGGKQALETVQRLLPVLCQAHGLTPEQVVAIASNIGGKQALETVQALLPVLCQAHGLTPEQVVAIASHDGGKQALETVQRLLPVLCQAHGLTPEQVVAIASNIGGKQALETVQALLPVLCQAHGLTPQQVVAIASNNGGKQALETVQRLLPVLCQAHGLTPEQVVAIASNIGGKQALETVQALLPVLCQAHGLTPQQVVAIASNGGGKQALETVQRLLPVLCQAHGLTPEQVVAIASNIGGKQALETVQALLPVLCQAHGLTPQQVVAIASNGGGKQALETVQRLLPVLCQAHGLTPEQVVAIASHDGGKQALETVQRLLPVLCQAHGLTPQQVVAIASNGGGRPALE

SEQ ID NO: 219 - protein, 530 aa, Artificial Sequence
  Synthetic Construct
LTPEQVVAIASHDGGKQALETVQRLLPVLCQAHGLTPQQVVAIASNGGGKQALETVQRLLPVLCQAHGLTPEQVVAIASHDGGKQALETVQRLLPVLCQAHGLTPEQVVAIASNIGGKQALETVQALLPVLCQAHGLTPQQVVAIASNNGGKQALETVQRLLPVLCQAHGLTPEQVVAIASHDGGKQALETVQRLLPVLCQAHGLTPQQVVAIASNGGGKQALETVQRLLPVLCQAHGLTPQQVVAIASNNGGKQALETVQRLLPVLCQAHGLTPQQVVAIASNNGGKQALETVQRLLPVLCQAHGLTPQQVVAIASNGGGKQALETVQRLLPVLCQAHGLTPEQVVAIASNIGGKQALETVQALLPVLCQAHGLTPEQVVAIASHDGGKQALETVQRLLPVLCQAHGLTPEQVVAIASNIGGKQALETVQALLPVLCQAHGLTPEQVVAIASHDGGKQALETVQRLLPVLCQAHGLTPQQVVAIASNNGGKQALETVQRLLPVLCQAHGLTPQQVVAIASNGGGRPALE

SEQ ID NO: 220 - protein, 530 aa, Artificial Sequence
  Synthetic Construct
LTPQQVVAIASNNGGKQALETVQRLLPVLCQAHGLTPQQVVAIASNGGGKQALETVQRLLPVLCQAHGLTPQQVVAIASNNGGKQALETVQRLLPVLCQAHGLTPQQVVAIASNGGGKQALETVQRLLPVLCQAHGLTPQQVVAIASNGGGKQALETVQRLLPVLCQAHGLTPQQVVAIASNGGGKQALETVQRLLPVLCQAHGLTPQQVVAIASNNGGKQALETVQRLLPVLCQAHGLTPEQVVAIASNIGGKQALETVQALLPVLCQAHGLTPQQVVAIASNNGGKQALETVQRLLPVLCQAHGLTPEQVVAIASHDGGKQALETVQRLLPVLCQAHGLTPEQVVAIASHDGGKQALETVQRLLPVLCQAHGLTPEQVVAIASNIGGKQALETVQALLPVLCQAHGLTPQQVVAIASNGGGKQALETVQRLLPVLCQAHGLTPEQVVAIASHDGGKQALETVQRLLPVLCQAHGLTPEQVVAIASNIGGKQALETVQALLPVLCQAHGLTPQQVVAIASNGGGRPALE

SEQ ID NO: 221 - protein, 539 aa, Artificial Sequence
  Synthetic Construct
NPQRSTVWYLTPQQVVAIASNNGGKQALETVQRLLPVLCQAHGLTPQQVVAIASNGGGKQALETVQRLLPVLCQAHGLTPQQVVAIASNNGGKQALETVQRLLPVLCQAHGLTPQQVVAIASNNGGKQALETVQRLLPVLCQAHGLTPEQVVAIASHDGGKQALETVQRLLPVLCQAHGLTPEQVVAIASHDGGKQALETVQRLLPVLCQAHGLTPQQVVAIASNGGGKQALETVQRLLPVLCQAHGLTPQQVVAIASNGGGKQALETVQRLLPVLCQAHGLTPQQVVAIASNGGGKQALETVQRLLPVLCQAHGLTPQQVVAIASNGGGKQALETVQRLLPVLCQAHGLTPQQVVAIASNNGGKQALETVQRLLPVLCQAHGLTPQQVVAIASNNGGKQALETVQRLLPVLCQAHGLTPQQVVAIASNNGGKQALETVQRLLPVLCQAHGLTPQQVVAIASNGGGKQALETVQRLLPVLCQAHGLTPQQVVAIASNNGGKQALETVQRLLPVLCQAHGLTPQQVVAIASNGGGRPALE

SEQ ID NO: 222 - protein, 530 aa, Artificial Sequence
  Synthetic Construct
LTPEQVVAIASHDGGKQALETVQRLLPVLCQAHGLTPEQVVAIASHDGGKQALETVQRLLPVLCQAHGLTPEQVVAIASHDGGKQALETVQRLLPVLCQAHGLTPEQVVAIASNIGGKQALETVQALLPVLCQAHGLTPEQVVAIASHDGGKQALETVQRLLPVLCQAHGLTPEQVVAIASHDGGKQALETVQRLLPVLCQAHGLTPEQVVAIASHDGGKQALETVQRLLPVLCQAHGLTPQQVVAIASNNGGKQALETVQRLLPVLCQAHGLTPEQVVAIASNIGGKQALETVQALLPVLCQAHGLTPQQVVAIASNNGGKQALETVQRLLPVLCQAHGLTPQQVVAIASNNGGKQALETVQRLLPVLCQAHGLTPQQVVAIASNGGGKQALETVQRLLPVLCQAHGLTPEQVVAIASHDGGKQALETVQRLLPVLCQAHGLTPQQVVAIASNNGGKQALETVQRLLPVLCQAHGLTPEQVVAIASHDGGKQALETVQRLLPVLCQAHGLTPQQVVAIASNGGGRPALE

SEQ ID NO: 223 - protein, 530 aa, Artificial Sequence
  Synthetic Construct
LTPQQVVAIASNNGGKQALETVQRLLPVLCQAHGLTPQQVVAIASNNGGKQALETVQRLLPVLCQAHGLTPQQVVAIASNNGGKQALETVQRLLPVLCQAHGLTPEQVVAIASNIGGKQALETVQALLPVLCQAHGLTPQQVVAIASNNGGKQALETVQRLLPVLCQAHGLTPEQVVAIASNIGGKQALETVQALLPVLCQAHGLTPQQVVAIASNGGGKQALETVQRLLPVLCQAHGLTPEQVVAIASHDGGKQALETVQRLLPVLCQAHGLTPQQVVAIASNGGGKQALETVQRLLPVLCQAHGLTPEQVVAIASHDGGKQALETVQRLLPVLCQAHGLTPQQVVAIASNGGGKQALETVQRLLPVLCQAHGLTPQQVVAIASNNGGKQALETVQRLLPVLCQAHGLTPEQVVAIASHDGGKQALETVQRLLPVLCQAHGLTPQQVVAIASNGGGKQALETVQRLLPVLCQAHGLTPQQVVAIASNGGGKQALETVQRLLPVLCQAHGLTPQQVVAIASNGGGRPALE

SEQ ID NO: 224 - protein, 530 aa, Artificial Sequence
  Synthetic Construct
LTPQQVVAIASNGGGKQALETVQRLLPVLCQAHGLTPEQVVAIASHDGGKQALETVQRLLPVLCQAHGLTPEQVVAIASHDGGKQALETVQRLLPVLCQAHGLTPQQVVAIASNGGGKQALETVQRLLPVLCQAHGLTPEQVVAIASHDGGKQALETVQRLLPVLCQAHGLTPEQVVAIASHDGGKQALETVQRLLPVLCQAHGLTPQQVVAIASNGGGKQALETVQRLLPVLCQAHGLTPEQVVAIASNIGGKQALETVQALLPVLCQAHGLTPEQVVAIASHDGGKQALETVQRLLPVLCQAHGLTPQQVVAIASNGGGKQALETVQRLLPVLCQAHGLTPEQVVAIASHDGGKQALETVQRLLPVLCQAHGLTPEQVVAIASNIGGKQALETVQALLPVLCQAHGLTPEQVVAIASHDGGKQALETVQRLLPVLCQAHGLTPEQVVAIASHDGGKQALETVQRLLPVLCQAHGLTPEQVVAIASNIGGKQALETVQALLPVLCQAHGLTPQQVVAIASNGGGRPALE

SEQ ID NO: 225 - protein, 530 aa, Artificial Sequence
  Synthetic Construct
LTPQQVVAIASNGGGKQALETVQRLLPVLCQAHGLTPQQVVAIASNNGGKQALETVQRLLPVLCQAHGLTPEQVVAIASHDGGKQALETVQRLLPVLCQAHGLTPQQVVAIASNGGGKQALETVQRLLPVLCQAHGLTPEQVVAIASHDGGKQALETVQRLLPVLCQAHGLTPQQVVAIASNGGGKQALETVQRLLPVLCQAHGLTPQQVVAIASNGGGKQALETVQRLLPVLCQAHGLTPEQVVAIASNIGGKQALETVQALLPVLCQAHGLTPEQVVAIASHDGGKQALETVQRLLPVLCQAHGLTPEQVVAIASHDGGKQALETVQRLLPVLCQAHGLTPQQVVAIASNGGGKQALETVQRLLPVLCQAHGLTPQQVVAIASNNGGKQALETVQRLLPVLCQAHGLTPQQVVAIASNGGGKQALETVQRLLPVLCQAHGLTPEQVVAIASNIGGKQALETVQALLPVLCQAHGLTPEQVVAIASHDGGKQALETVQRLLPVLCQAHGLTPQQVVAIASNGGGRPALE

SEQ ID NO: 226 - protein, 135 aa, Homo sapien
CPYSNPSLCSGGGGSELPTQGTFSNVSTNVSPAKPTTTACPYSNPSLCSGGGGSPAPRPPTPAPTIASQPLSLRPEACRPAAGGAVHTRGLDFACDIYIWAPLAGTCGVLLLSLVITLYCNHRNRRRVCKCPRPW

SEQ ID NO: 227 - protein, 19 aa, Artificial Sequence
  Synthetic Construct
CGSGSGLEEKKGNYVVTDH

SEQ ID NO: 228 - DNA, 804 bp, Artificial Sequence
  Synthetic Construct
atggctctgcccgtcaccgctctgctgctgcccctggctctgctgctgcacgctgctcgccctgatgtggtcatgactcagtctcccctgtctctgcccgtcaccctgggacagcccgccagcatctcctgcaagagctcccagagcctgctgtactccaacggcaagacctatctgaattggttccagcagagacccggccagagccctcggagactgatctaccaggtgtctaagctggacagcggcgtgcctgatcgcttctctggaagcggatccggaaccgactttacactgaagatcagccgggtggaggcagaggacgtgggcgtgtactattgcggccaggatacccacttcccactgacatttggcggcggcaccaaggtggagatcaagggaggaggaggaagcggaggaggaggaagcggcggcggcggctctggcggcggcggcagccaggtgcagctggtgcagagcggagcagaggtgaagaagcctggcgcctccgtgaaggtgtcttgtaaggccagcggctacacattcaccgattatacactgcactgggtgcggcaggcccctggccagggactggagtggatgggaggaatctggcctatcaccggaggaaccacatacaaccagaagtttaagggcagagtgacaatgaccagggacacatctaccagcacagtgtatatggagctgtctagcctgcgctccgaggatacagccgtgtactattgcgccagaggcgaggcacagggatcttggggacagggcaccctggtgacagtgtcctct

SEQ ID NO: 229 - DNA, 807 bp, Artificial Sequence
  Synthetic Construct
atggctctgcccgtcaccgctctgctgctgccactggccctgctgctgcacgcagcaaggcctcaggtgaccctgaaggagagcggccctgtgctgctgaagccaacagagaccctgacactgacctgcacagtgtctggcttcagcctgtccaacccccggatgggcgtgagctggatcagacagccccctggcaaggccctggagtggttcgcccacatcttttctaccgatgagaagagcctgaagctgtccctgagatctaggctgaccctgagcaaggacacatctaagagccaggtggtgctgaccatgacaaacatggcccctgtggactccgccacatactattgcgccagagacagctccaattacgagggctatttcgacttttggggccagggcaccctggtgacagtgtctagcggcggaggaggatccggaggaggaggatctggcggcggcggctccggcggcggcggctccgaggtggtgctgacccagagccctgccacactgtccgtgtctccaggcgagagagccaccctgtcttgtagggccagccagtccgtgcgcagcaatctggcctggtaccagcagaagtccggccaggccccaagactgctgatctatggctccaccatcagggccacaggagtgccagcacgcttctctggaagcggatccggcacagagtttaccctgacaatctcctctctgcagtccgaggatttcgccgtgtactattgccagcagtactctgactggcccttcacctttggccctggcacaaaggtggatatcaag

SEQ ID NO: 230 - DNA, 807 bp, Artificial Sequence
  Synthetic Construct
atggctctgcccgtcaccgctctgctgctgccactggccctgctgctgcacgcagcaaggccacaggtgaccctgaaggagtccggccccgtgctggtgaagcctacagagaccctgacactgacctgcacagtgtccggcttctctctgagcaacgcccgcatgggcgtgtcttggatcaggcagccccctggcaaggccctggagtggctggcccacatcttttccaccgacgagaagtctatccggagaagcctgcgctccaggctgaccctgagcaaggatacatccaagtctcaggtggtgctgaccatgacaaacatggaccccgtggataccgccacatacttctgcgccagagacagctccaattacgagggctattttgattactggggccagggcaccctggtgacagtgtctagcggaggaggaggaagcggaggaggaggatctggcggcggcggctctggcggcggcggcagcgaggtggtcatgacccagagcccagccacactgagcgtgtcccctggcgagagggtgaccctgtcctgtagggcatctcagagcgtgtcctctaacttcgcctggtatcagcagagaccaggccaggcaccaaggctgctgctgtacggagcaaccacaagagccacaggactgcccggcaggttttccggatctggaagcggcaccgagaatatcctgacaatcagctccctgcagtctgaggacttcgccatctatttttgccagcagtacaaggattggccattcacctttggccccggcagcaaggtggacatcaag

SEQ ID NO: 231 - DNA, 807 bp, Artificial Sequence
  Synthetic Construct
atggctctgcccgtcaccgctctgctgctgccactggccctgctgctgcacgcagcaagacctcaggtgaccctgaaggagtccggccctgtgctggtgaagccaacagagaccctgacactgacctgcacagtgtctggcttcagcctgtccaacgcaaggatgggcgtgagctggatcaggcagccccctggcaaggccctggagtggctgggccacatctttagcaccgacgagaagtcttacagcacatccctgagaggcaggatcaccatctctaaggatacaagcagaggcctggtggtgctgaccctgacaaacatggaccccgtggataccgccacatactattgcgccagggacagctccaattacgagggctatttcgatttttggggccctggcttcctggtgaccgtgtctagcggcggcggcggctctggaggaggaggaagcggaggaggaggatccggcggcggcggctctgagatcgtgatgacccagtcccctgccacactgtctgtgagcccaggcgagagagccaccctgtcttgtagggtgtcccagtctatcggcgccaatctggcctggtaccagcagaagttcggccaggccccaaggctgctgatctatggagcatccaccagagccacaggaatccccgtgaggttctccggaggaggatctggaaccgagtttaccctgacaatctcctctctgcagagcgaggactttgccatctactcctgccagcagtacatctattggcccttcacatttggccctggcaccacagtggatatcaag

SEQ ID NO: 232 - DNA, 807 bp, Artificial Sequence
  Synthetic Construct
atggctctgcccgtcaccgctctgctgctgccactggccctgctgctgcacgcagcaagaccacaggtgaccctgaaggagagcggacccgtgctggtgaagcctacagagaccctgacactgacctgcacagtgagcggcttctccctgaacaatgcaaggatgggcgtgtcctggatcaggcagccccctggcaaggccctggagtggttcgcccacatctttagcaccgacgagaagtcctttcgcacatctctgagaagcaggctgaccctgagcaaggatacaagcaagtcccaggtggtgctgaccatgacaaacatggaccccgtggataccgccacatactattgcgccagagacagctccaattacgagggctatttcgattactggggccagggcatcctggtgaccgtgtctagcggcggcggcggctctggaggaggaggaagcggaggaggaggatccggcggcggcggctctgagatcgtgatgacccagtctcccgccacactgtctgtgagccctggcgagagagccacactgagctgtagggcctcccagtctgtgagcaacaatctggcctggtatcagcagaagccaggccaggcaccaaggctgctgatctacggagcatccaccagagccacaggagtgccagcaaggttctccggatctgacagcggcaccgagtttagcctgacaatctcctctctgcagtccgaggacttcgccgtgtatttttgccagcagtacaaggattggccattcacctttggccccggcacaaaggtggagatcaag

SEQ ID NO: 233 - DNA, 819 bp, Artificial Sequence
  Synthetic Construct
atggctctgcccgtcaccgctctgctgctgccactggccctgctgctgcacgcagcaaggccagaggtgaacctggtggagtccggcggcggcctggtgaagcctggcggatccctgaggctgtcttgcgaggcaagcggcttcaccttcagctacgcctggatgtcctgggtgcgccaggcccccggcaagggactggagtgggtgggacggatcaagtccatcgcagacggaggagcaaccgattacgcagcccctgtgagaaacaggttcacaatctccagagacgattctaggaataccctgtatctggagatgcactctctgaagacagaggacaccgccgtgtactattgcaccacaatccctggcaacgacgcctttgatatgtggggccagggcacaatggtgaccgtgagctccggcggcggcggctctggaggaggaggaagcggaggaggaggaagcgggggcggcggctctgacatcgtgctgacacagtccccactgtccctgtctgtgacccccggcgagcctgcaagcatctcctgtagatctagccagagcctgctgtactccaacggcaagaattatctggattggttcctgcacaagccaggccagtctccccagctgctgatctacctgggatctaatagggcaagcggagtgccagaccggttctctggaagcggatccggcatcgacttcatcctgaagatcagcagggtggaggccgaggatgtgggcgtgtactattgcatgcaggcccagcagacacccatcaccttcggccagggcacaagactggagatcaag

SEQ ID NO: 234 - DNA, 819 bp, Artificial Sequence
  Synthetic Construct
atggctctgcccgtcaccgctctgctgctgccactggccctgctgctgcacgcagcaaggccagaggtgaacctggtggagtccggcggcggcctggtgaagcctggcggatccctgaggctgtcttgcgaggcaagcggcttcaccttcagctacgcctggatgtcctgggtgcgccaggcccccggcaagggactggagtgggtgggccggatcaagtccatcaccgacggaggcgtgatcgattacgcagcacctgtgagaaacaggtgcacaatctccagagacgattctaggaataccctgtatctggagatgcactctctgaagacagaggacaccgccgtgtactattgtaccacaatccctggcaacgacgatttcgatatgtggggccagggcagaatggtgaccgtgagctccggcggcggcggctctggaggaggaggaagcggaggaggaggaagcgggggcggcggctctgacatcgtgctgacacagtccccactgtccctgtctgtgacccccggcgagcctgcaagcatctcctgtaggtctagccagagcctgctgtactccaacggcaagaattatctggattggtttctgcacaagccaggccagtctccccagctgctgatctacctgggatctaatagggcaagcggagtgccagaccggttctctggaagcggatccggcatcgacttcatcctgaagatcagccgcgtggaggcagaggacgtgggcgtgtactattgcatgcaggcccagcagacacccatcaccttcggccagggcacaagactggagatcaag

SEQ ID NO: 235 - DNA, 816 bp, Artificial Sequence
  Synthetic Construct
atggctctgcccgtcaccgctctgctgctgccactggccctgctgctgcacgcagcaaggccagaggtgcagctggtggagtcttggggcgtgctggtgaagcctggcggatctctgaggctgagctgcgcagcatccggcttcatctttaacaatgcctggatgtcctgggtgcgccaggcccccggcaagggactggagtggatcggccggatcaagagcaagtccgacggaggaaccacagattacgcagcacctgtgaaggaccgcttcacaatctctcgggacgatagcaaggataccctgtatctgcagatgaacggcctgaagacagaggacaccgccgtgtacttctgcaccacagcccctggcggcccttttgattattggggccagggcacactggtgaccgtgagctccggaggaggaggaagcggcggaggaggcagcggcggcggcggctctggcggcggcggcagcgacatcgtgctgacacagagccctctgtccctgccagtgacccccggcgagcctgcctctatcagctgtcgctctagccagagcctgctgcaccgggacggcttcaattacctggattggtttctgcagaagccaggccagtccccccagctgctgatctatctggcctcctctagagcctctggcgtgccagacaggttctccggctctgacagcggcacagacttcaccctgaagatcagcagagtggaggccgaggatgtgggcgtgtactattgcatgcaggccctgcagacacccatcaccttcggccagggcacaagactggagatcaag

SEQ ID NO: 236 - DNA, 813 bp, Artificial Sequence
  Synthetic Construct
atggctctgcccgtcaccgctctgctgctgccactggccctgctgctgcacgcagcaaggcctgaggtgcagctggtggagagcggcggcggcctggtgaagcctggcggatccctgaggctgtcttgcgaggcaagcggcttcacctttagcgacgcatggatgtcctgggtgcgccaggcccctggcaagggactggagtgggtgggacggatcaagagcaagacagacggcggcaccacagattacgtggtgccactgaacggccgcttcatcatctcccgcgacgattctcggaataccctgtatctgcagctgaacaatctgaagacagaggataccgccgtgtactattgcaccacagtgccaggctcctacggctattggggccagggcacactggtgaccgtgagctccggcggcggcggctctggaggaggaggaagcggaggaggaggaagcgggggcggcggctctgacatcgtgatgacacagtctccactgagcctgccagtgacccctggcgagccagcctccatctcttgtcgctctagccagagcctgctgcacaacaagcggaacaattacctggattggtttctgcagaagcctggccagtcccctcagctgctgatctatctggccagcaatagagcctccggagtgccagacaggttctctggaggaggaagcggaacagacttcaccctgaagatcagcagagtggaggccgaggacgtgggcgtgtactattgcatgcaggcccagcagacacctatcaccttcggccagggcacaagactggagatcaag

SEQ ID NO: 237 - DNA, 837 bp, Artificial Sequence
  Synthetic Construct
atggctctgcccgtcaccgctctgctgctgcctctggccctgctgctgcacgcagcaaggccacaggtgcagctggtgcagtccggagcagaggtgaagaagcctggcagctccgtgaaggtgagctgcaaggcctccggcgacacattctctagcaacgcaatcagctgggtgcgccaggcccctggccagggactggagtggatgggcgtgatcatccctatcttcggcaccgccgactatgcccagaagtttcagggccgggtgacaatcaccgccgatgagtctacaagcaccgcctacatggagctgtcctctctgagatccgaggacacagccgtgtactattgtgccaggcacacctatcacgagtacgcaggaggatactatggaggagcaatggatccttggggacagggcacactggtgaccgtgagctccggcggcggcggctctggaggaggaggaagcggaggaggaggaagcgggggcggcggctctgagctgcagagcgtgctgacccagccaccttccgcctctggaacaccaggccagagggtgaccatcagctgctccggatctagctccaacatcggctccaattacgtgtattggtaccagcagctgccaggcacagcccccaagatcctgatctaccgcaacaatcagcggccttctggcgtgccagatagattctctggcagcaagtccggcacctctgccagcctggcaatctccggcctgaggtctgaggacgaggccgattactattgcgccgcctgggacgataacctgagcggctgggtgtttggcacaggcaccaagctgacagtgctg

SEQ ID NO: 238 - DNA, 1476 bp, Artificial Sequence
  Synthetic Construct
atggctctgcccgtcaccgctctgctgctgcccctggctctgctgctgcacgctgctcgccctgatgtggtcatgactcagtctcccctgtctctgcccgtcaccctgggacagcccgccagcatctcctgcaagagctcccagagcctgctgtactccaacggcaagacctatctgaattggttccagcagagacccggccagagccctcggagactgatctaccaggtgtctaagctggacagcggcgtgcctgatcgcttctctggaagcggatccggaaccgactttacactgaagatcagccgggtggaggcagaggacgtgggcgtgtactattgcggccaggatacccacttcccactgacatttggcggcggcaccaaggtggagatcaagggaggaggaggaagcggaggaggaggaagcggcggcggcggctctggcggcggcggcagccaggtgcagctggtgcagagcggagcagaggtgaagaagcctggcgcctccgtgaaggtgtcttgtaaggccagcggctacacattcaccgattatacactgcactgggtgcggcaggcccctggccagggactggagtggatgggaggaatctggcctatcaccggaggaaccacatacaaccagaagtttaagggcagagtgacaatgaccagggacacatctaccagcacagtgtatatggagctgtctagcctgcgctccgaggatacagccgtgtactattgcgccagaggcgaggcacagggatcttggggacagggcaccctggtgacagtgtcctctaccacaaccccagcaccaagaccacctacccctgcaccaacaatcgcctcccagcctctgtctctgcgcccagaggcatgtaggccagcagcaggaggagcagtgcacaccaggggcctggactttgcctgcgatatctacatctgggcaccactggcaggaacatgtggcgtgctgctgctgagcctggtcatcaccctgtactgcaagcgcggccggaagaagctgctgtatatcttcaagcagcccttcatgagacccgtgcagacaacccaggaggaggacggctgctcctgtaggttcccagaagaagaggagggcggctgtgagctgagagtgaagttttccaggtctgccgatgcaccagcataccagcagggacagaatcagctgtataacgagctgaatctgggcaggcgcgaggagtatgacgtgctggataagaggagaggaagggaccctgagatgggaggcaagcctaggcgcaagaacccacaggagggcctgtacaatgagctgcagaaggataagatggccgaggcctattccgagatcggcatgaagggcgagcggagaaggggcaagggccacgacgggctgtaccagggactgtcaaccgctaccaaggatacttacgacgccctgcatatgcaggcactgcctccaaggtga

SEQ ID NO: 239 - DNA, 1479 bp, Artificial Sequence
  Synthetic Construct
atggctctgcccgtcaccgctctgctgctgccactggccctgctgctgcacgcagcaaggcctcaggtgaccctgaaggagagcggccctgtgctgctgaagccaacagagaccctgacactgacctgcacagtgtctggcttcagcctgtccaacccccggatgggcgtgagctggatcagacagccccctggcaaggccctggagtggttcgcccacatcttttctaccgatgagaagagcctgaagctgtccctgagatctaggctgaccctgagcaaggacacatctaagagccaggtggtgctgaccatgacaaacatggcccctgtggactccgccacatactattgcgccagagacagctccaattacgagggctatttcgacttttggggccagggcaccctggtgacagtgtctagcggcggaggaggatccggaggaggaggatctggcggcggcggctccggcggcggcggctccgaggtggtgctgacccagagccctgccacactgtccgtgtctccaggcgagagagccaccctgtcttgtagggccagccagtccgtgcgcagcaatctggcctggtaccagcagaagtccggccaggccccaagactgctgatctatggctccaccatcagggccacaggagtgccagcacgcttctctggaagcggatccggcacagagtttaccctgacaatctcctctctgcagtccgaggatttcgccgtgtactattgccagcagtactctgactggcccttcacctttggccctggcacaaaggtggatatcaagaccacaacccctgcaccaaggccaccaaccccagcacctacaatcgcaagccagccactgtccctgagacccgaggcctgtaggcctgcagcaggaggagcagtgcacacccgcggcctggactttgcctgcgatatctatatctgggcaccactggcaggaacctgtggcgtgctgctgctgagcctggtcatcaccctgtactgcaagcgcggccggaagaagctgctgtatatcttcaagcagcccttcatgcggcccgtgcagacaacccaggaggaggatggctgctcctgtagattccctgaggaggaggagggaggatgtgagctgagggtgaagttttctcggagcgccgacgcaccagcataccagcagggacagaaccagctgtataacgagctgaatctgggccggagagaggagtacgacgtgctggataagaggaggggaagagacccagagatgggaggcaagccacggagaaagaacccccaggagggcctgtacaatgagctgcagaaggataagatggccgaggcctattctgagatcggcatgaagggagagaggcgccggggcaagggacacgacggactgtaccagggactgtccaccgcaacaaaggacacctatgatgccctgcatatgcaggcactgcctccaaggtga

SEQ ID NO: 240 - DNA, 1479 bp, Artificial Sequence
  Synthetic Construct
atggctctgcccgtcaccgctctgctgctgccactggccctgctgctgcacgcagcaaggccacaggtgaccctgaaggagtccggccccgtgctggtgaagcctacagagaccctgacactgacctgcacagtgtccggcttctctctgagcaacgcccgcatgggcgtgtcttggatcaggcagccccctggcaaggccctggagtggctggcccacatcttttccaccgacgagaagtctatccggagaagcctgcgctccaggctgaccctgagcaaggatacatccaagtctcaggtggtgctgaccatgacaaacatggaccccgtggataccgccacatacttctgcgccagagacagctccaattacgagggctattttgattactggggccagggcaccctggtgacagtgtctagcggaggaggaggaagcggaggaggaggatctggcggcggcggctctggcggcggcggcagcgaggtggtcatgacccagagcccagccacactgagcgtgtcccctggcgagagggtgaccctgtcctgtagggcatctcagagcgtgtcctctaacttcgcctggtatcagcagagaccaggccaggcaccaaggctgctgctgtacggagcaaccacaagagccacaggactgcccggcaggttttccggatctggaagcggcaccgagaatatcctgacaatcagctccctgcagtctgaggacttcgccatctatttttgccagcagtacaaggattggccattcacctttggccccggcagcaaggtggacatcaagaccacaacccctgcaccaagaccaccaaccccagcacctacaatcgcctctcagcctctgagcctgcgcccagaggcatgtaggccagcagcaggaggagcagtgcacacaaggggcctggacttcgcctgcgatatctatatctgggcacctctggcaggaacctgtggcgtgctgctgctgagcctggtcatcaccctgtattgcaagagaggcaggaagaagctgctgtacatcttcaagcagccttttatgcgcccagtgcagacaacccaggaggaggacggctgcagctgtcggttccctgaagaggaggagggcggctgtgagctgagagtgaagttttccaggtctgccgatgccccagcctatcagcagggccagaatcagctgtacaacgagctgaatctgggcaggcgcgaggagtacgacgtgctggataagaggagaggaagggatccagagatgggaggcaagcctaggcgcaagaacccacaggagggcctgtataatgagctgcagaaggacaagatggccgaggcctactccgagatcggcatgaagggagagcggagaaggggcaagggacacgatggcctgtatcagggcctgtctaccgccacaaaggacacctacgatgccctgcatatgcaggcactgcctccaaggtga

SEQ ID NO: 241 - DNA, 1479 bp, Artificial Sequence
  Synthetic Construct
atggctctgcccgtcaccgctctgctgctgccactggccctgctgctgcacgcagcaagacctcaggtgaccctgaaggagtccggccctgtgctggtgaagccaacagagaccctgacactgacctgcacagtgtctggcttcagcctgtccaacgcaaggatgggcgtgagctggatcaggcagccccctggcaaggccctggagtggctgggccacatctttagcaccgacgagaagtcttacagcacatccctgagaggcaggatcaccatctctaaggatacaagcagaggcctggtggtgctgaccctgacaaacatggaccccgtggataccgccacatactattgcgccagggacagctccaattacgagggctatttcgatttttggggccctggcttcctggtgaccgtgtctagcggcggcggcggctctggaggaggaggaagcggaggaggaggatccggcggcggcggctctgagatcgtgatgacccagtcccctgccacactgtctgtgagcccaggcgagagagccaccctgtcttgtagggtgtcccagtctatcggcgccaatctggcctggtaccagcagaagttcggccaggccccaaggctgctgatctatggagcatccaccagagccacaggaatccccgtgaggttctccggaggaggatctggaaccgagtttaccctgacaatctcctctctgcagagcgaggactttgccatctactcctgccagcagtacatctattggcccttcacatttggccctggcaccacagtggatatcaagaccacaacccctgcaccaaggccaccaaccccagcacctacaatcgcaagccagccactgtccctgagaccagaggcatgtaggcctgcagcaggaggagccgtgcacaccagaggcctggactttgcctgcgatatctatatctgggcaccactggcaggaacctgtggcgtgctgctgctgagcctggtcatcaccctgtactgcaagcgcggccggaagaagctgctgtatatcttcaagcagcccttcatgcgccccgtgcagacaacccaggaggaggacggctgcagctgtcggttccctgaagaggaggagggaggatgtgagctgagggtgaagtttagccggtccgccgatgcaccagcataccagcagggccagaaccagctgtataacgagctgaatctgggccggagagaggagtacgacgtgctggataagaggaggggaagagacccagagatgggaggcaagccacggagaaagaacccccaggagggcctgtacaatgagctgcagaaggacaagatggccgaggcctatagcgagatcggcatgaagggagagaggcgccggggcaagggacacgatggcctgtaccagggcctgtccaccgccacaaaggacacctatgatgccctgcatatgcaggcactgcctccaaggtga

SEQ ID NO: 242 - DNA, 1479 bp, Artificial Sequence
  Synthetic Construct
atggctctgcccgtcaccgctctgctgctgccactggccctgctgctgcacgcagcaagaccacaggtgaccctgaaggagagcggacccgtgctggtgaagcctacagagaccctgacactgacctgcacagtgagcggcttctccctgaacaatgcaaggatgggcgtgtcctggatcaggcagccccctggcaaggccctggagtggttcgcccacatctttagcaccgacgagaagtcctttcgcacatctctgagaagcaggctgaccctgagcaaggatacaagcaagtcccaggtggtgctgaccatgacaaacatggaccccgtggataccgccacatactattgcgccagagacagctccaattacgagggctatttcgattactggggccagggcatcctggtgaccgtgtctagcggcggcggcggctctggaggaggaggaagcggaggaggaggatccggcggcggcggctctgagatcgtgatgacccagtctcccgccacactgtctgtgagccctggcgagagagccacactgagctgtagggcctcccagtctgtgagcaacaatctggcctggtatcagcagaagccaggccaggcaccaaggctgctgatctacggagcatccaccagagccacaggagtgccagcaaggttctccggatctgacagcggcaccgagtttagcctgacaatctcctctctgcagtccgaggacttcgccgtgtatttttgccagcagtacaaggattggccattcacctttggccccggcacaaaggtggagatcaagaccacaacccctgcaccaagaccaccaaccccagcacctacaatcgcatcccagcctctgtctctgagaccagaggcatgtaggccagcagcaggaggagcagtgcacaccaggggcctggactttgcctgcgatatctatatctgggcacctctggcaggaacctgtggcgtgctgctgctgagcctggtcatcaccctgtattgcaagcgcggccggaagaagctgctgtacatcttcaagcagccttttatgcgcccagtgcagacaacccaggaggaggacggctgctcctgtcggttccctgaagaggaggagggaggatgtgagctgagggtgaagttttcccggtctgccgatgccccagcctatcagcagggccagaaccagctgtacaacgagctgaatctgggccggagagaggagtacgacgtgctggataagaggaggggaagagatccagagatgggaggcaagcctcggagaaagaacccacaggagggcctgtataatgagctgcagaaggacaagatggccgaggcctactccgagatcggcatgaagggagagaggcgccggggcaagggacacgatggcctgtatcagggcctgtctaccgccacaaaggacacctacgatgccctgcatatgcaggcactgcctccaaggtga

SEQ ID NO: 243 - DNA, 1491 bp, Artificial Sequence
  Synthetic Construct
atggctctgcccgtcaccgctctgctgctgccactggccctgctgctgcacgcagcaaggccagaggtgaacctggtggagtccggcggcggcctggtgaagcctggcggatccctgaggctgtcttgcgaggcaagcggcttcaccttcagctacgcctggatgtcctgggtgcgccaggcccccggcaagggactggagtgggtgggacggatcaagtccatcgcagacggaggagcaaccgattacgcagcccctgtgagaaacaggttcacaatctccagagacgattctaggaataccctgtatctggagatgcactctctgaagacagaggacaccgccgtgtactattgcaccacaatccctggcaacgacgcctttgatatgtggggccagggcacaatggtgaccgtgagctccggcggcggcggctctggaggaggaggaagcggaggaggaggaagcgggggcggcggctctgacatcgtgctgacacagtccccactgtccctgtctgtgacccccggcgagcctgcaagcatctcctgtagatctagccagagcctgctgtactccaacggcaagaattatctggattggttcctgcacaagccaggccagtctccccagctgctgatctacctgggatctaatagggcaagcggagtgccagaccggttctctggaagcggatccggcatcgacttcatcctgaagatcagcagggtggaggccgaggatgtgggcgtgtactattgcatgcaggcccagcagacacccatcaccttcggccagggcacaagactggagatcaagaccacaaccccagcaccaaggccacctacacctgcaccaaccatcgcatcccagccactgtctctgaggcctgaggcatgtcggccagcagcaggaggagcagtgcacacccgcggcctggactttgcctgcgatatctacatctgggcaccactggcaggaacatgtggcgtgctgctgctgagcctggtcatcaccctgtactgcaagcgcggccggaagaagctgctgtatatcttcaagcagccttttatgagaccagtgcagacaacccaggaggaggacggctgctcctgtaggttccctgaagaggaggagggcggctgtgagctgagagtgaagttttctaggagcgccgatgcaccagcataccagcagggacagaatcagctgtataacgagctgaatctgggccggagagaggagtatgacgtgctggataagaggaggggaagggaccctgagatgggaggcaagccccggagaaagaaccctcaggagggcctgtacaatgagctgcagaaggacaagatggccgaggcctatagcgagatcggcatgaagggagagaggcgccggggcaagggacacgatggcctgtaccagggcctgtccacagccaccaaggacacctatgatgccctgcatatgcaggcactgcctccaaggtga

SEQ ID NO: 244 - DNA, 1491 bp, Artificial Sequence
  Synthetic Construct
atggctctgcccgtcaccgctctgctgctgccactggccctgctgctgcacgcagcaaggccagaggtgaacctggtggagtccggcggcggcctggtgaagcctggcggatccctgaggctgtcttgcgaggcaagcggcttcaccttcagctacgcctggatgtcctgggtgcgccaggcccccggcaagggactggagtgggtgggccggatcaagtccatcaccgacggaggcgtgatcgattacgcagcacctgtgagaaacaggtgcacaatctccagagacgattctaggaataccctgtatctggagatgcactctctgaagacagaggacaccgccgtgtactattgtaccacaatccctggcaacgacgatttcgatatgtggggccagggcagaatggtgaccgtgagctccggcggcggcggctctggaggaggaggaagcggaggaggaggaagcgggggcggcggctctgacatcgtgctgacacagtccccactgtccctgtctgtgacccccggcgagcctgcaagcatctcctgtaggtctagccagagcctgctgtactccaacggcaagaattatctggattggtttctgcacaagccaggccagtctccccagctgctgatctacctgggatctaatagggcaagcggagtgccagaccggttctctggaagcggatccggcatcgacttcatcctgaagatcagccgcgtggaggcagaggacgtgggcgtgtactattgcatgcaggcccagcagacacccatcaccttcggccagggcacaagactggagatcaagaccacaaccccagcaccaaggccacctacacctgcaccaaccatcgcatcccagccactgtctctgaggcctgaggcatgtaggccagcagcaggaggagcagtgcacaccagaggcctggactttgcctgcgatatctacatctgggcaccactggcaggaacatgtggcgtgctgctgctgagcctggtcatcaccctgtactgcaagcgcggccggaagaagctgctgtatatcttcaagcagccttttatgagaccagtgcagacaacccaggaggaggacggctgctcctgtaggttccctgaagaggaggagggcggctgtgagctgagagtgaagttttctaggagcgccgatgcaccagcataccagcagggacagaatcagctgtataacgagctgaatctgggccggagagaggagtatgacgtgctggataagaggaggggaagggatcctgagatgggaggcaagccccggagaaagaaccctcaggagggcctgtacaatgagctgcagaaggacaagatggccgaggcctatagcgagatcggcatgaagggagagaggcgccggggcaagggacacgatggcctgtaccagggcctgtccacagccaccaaggacacctatgatgccctgcatatgcaggcactgcctccaaggtga

SEQ ID NO: 245 - DNA, 1488 bp, Artificial Sequence
  Synthetic Construct
atggctctgcccgtcaccgctctgctgctgccactggccctgctgctgcacgcagcaaggccagaggtgcagctggtggagtcttggggcgtgctggtgaagcctggcggatctctgaggctgagctgcgcagcatccggcttcatctttaacaatgcctggatgtcctgggtgcgccaggcccccggcaagggactggagtggatcggccggatcaagagcaagtccgacggaggaaccacagattacgcagcacctgtgaaggaccgcttcacaatctctcgggacgatagcaaggataccctgtatctgcagatgaacggcctgaagacagaggacaccgccgtgtacttctgcaccacagcccctggcggcccttttgattattggggccagggcacactggtgaccgtgagctccggaggaggaggaagcggcggaggaggcagcggcggcggcggctctggcggcggcggcagcgacatcgtgctgacacagagccctctgtccctgccagtgacccccggcgagcctgcctctatcagctgtcgctctagccagagcctgctgcaccgggacggcttcaattacctggattggtttctgcagaagccaggccagtccccccagctgctgatctatctggcctcctctagagcctctggcgtgccagacaggttctccggctctgacagcggcacagacttcaccctgaagatcagcagagtggaggccgaggatgtgggcgtgtactattgcatgcaggccctgcagacacccatcaccttcggccagggcacaagactggagatcaagaccacaaccccagcaccaaggccacctacacctgcaccaaccatcgcatcccagccactgtctctgagacctgaggcctgtaggccagcagcaggaggagcagtgcacaccaggggcctggactttgcctgcgatatctacatctgggcacctctggcaggaacatgtggcgtgctgctgctgagcctggtcatcaccctgtactgcaagagaggcaggaagaagctgctgtatatcttcaagcagccttttatgagaccagtgcagacaacccaggaggaggacggctgctcctgtaggttccctgaagaggaggagggaggatgtgagctgagggtgaagttttcccggtctgccgatgcaccagcataccagcagggacagaaccagctgtataacgagctgaatctgggccggagagaggagtacgacgtgctggataagaggcgcggcagagatccagagatgggcggcaagccccggagaaagaaccctcaggagggcctgtacaatgagctgcagaaggacaagatggccgaggcctatagcgagatcggcatgaagggagagaggcgccggggcaagggacacgatggcctgtaccagggcctgtccacagccaccaaggacacctatgatgccctgcatatgcaggcactgcctccaaggtga

SEQ ID NO: 246 - DNA, 1485 bp, Artificial Sequence
  Synthetic Construct
atggctctgcccgtcaccgctctgctgctgccactggccctgctgctgcacgcagcaaggcctgaggtgcagctggtggagagcggcggcggcctggtgaagcctggcggatccctgaggctgtcttgcgaggcaagcggcttcacctttagcgacgcatggatgtcctgggtgcgccaggcccctggcaagggactggagtgggtgggacggatcaagagcaagacagacggcggcaccacagattacgtggtgccactgaacggccgcttcatcatctcccgcgacgattctcggaataccctgtatctgcagctgaacaatctgaagacagaggataccgccgtgtactattgcaccacagtgccaggctcctacggctattggggccagggcacactggtgaccgtgagctccggcggcggcggctctggaggaggaggaagcggaggaggaggaagcgggggcggcggctctgacatcgtgatgacacagtctccactgagcctgccagtgacccctggcgagccagcctccatctcttgtcgctctagccagagcctgctgcacaacaagcggaacaattacctggattggtttctgcagaagcctggccagtcccctcagctgctgatctatctggccagcaatagagcctccggagtgccagacaggttctctggaggaggaagcggaacagacttcaccctgaagatcagcagagtggaggccgaggacgtgggcgtgtactattgcatgcaggcccagcagacacctatcaccttcggccagggcacaagactggagatcaagaccacaaccccagcaccaaggccacctacacctgcaccaaccatcgcctcccagcctctgtctctgagaccagaggcatgtaggccagcagcaggaggagcagtgcacaccaggggcctggactttgcctgcgatatctacatctgggcacctctggcaggaacatgtggcgtgctgctgctgagcctggtcatcaccctgtactgcaagagaggcaggaagaagctgctgtatatcttcaagcagcccttcatgagacccgtgcagacaacccaggaggaggacggctgctcttgtaggttcccagaagaggaggagggaggatgtgagctgagggtgaagtttagccggtccgccgatgcaccagcataccagcagggacagaaccagctgtataacgagctgaatctgggccggagagaggagtacgacgtgctggataagaggaggggaagggatccagagatgggaggcaagcctcggagaaagaacccacaggagggcctgtacaatgagctgcagaaggacaagatggccgaggcctattctgagatcggcatgaagggagagaggcgccggggcaagggacacgatggcctgtaccagggcctgagcacagccaccaaggacacctatgatgccctgcatatgcaggcactgcctccaaggtga

SEQ ID NO: 247 - DNA, 1508 bp, Artificial Sequence
  Synthetic Construct
atggctctgcccgtcaccgctctgctgctgcctctggccctgctgctgcacgcagcaaggccacaggtgcagctggtgcagtccggagcagaggtgaagaagcctggcagctccgtgaaggtgagctgcaaggcctccggcgacacattctctagcaacgcaatcagctgggtgcgccaggcccctggccagggactggagtggatgggcgtgatcatccctatcttcggcaccgccgactatgcccagaagtttcagggccgggtgacaatcaccgccgatgagtctacaagcaccgcctacatggagctgtcctctctgagatccgaggacacagccgtgtactattgtgccaggcacacctatcacgagtacgcaggaggatactatggaggagcaatggatccttggggacagggcacactggtgaccgtgagctccggcggcggcggctctggaggaggaggaagcggaggaggaggaagcgggggcggcggctctgagctgcagagcgtgctgacccagccaccttccgcctctggaacaccaggccagagggtgaccatcagctgctccggatctagctccaacatcggctccaattacgtgtattggtaccagcagctgccaggcacagcccccaagatcctgatctaccgcaacaatcagcggccttctggcgtgccagatagattctctggcagcaagtccggcacctctgccagcctggcaatctccggcctgaggtctgaggacgaggccgattactattgcgccgcctgggacgataacctgagcggctgggtgtttggcacaggcaccaagctgacagtgctgaccacaacccctgcaccaagaccaccaacaccagcacctaccatcgcaagccagccactgtccctgagacccgaggcctgtaggcctgcagcaggaggagcagtgcacaccaggggcctggactttgcctgcgatatctatatctgggcaccactggcaggaacatgtggcgtgctgctgctgagcctggtcatcaccctgtattgcaagagaggcaggaagaagctgctgtacatcttcaagcagccctttatgcgccctgtgcagacaacccaggaggaggacggctgcagctgtcggttcccagaagaggaggagggaggatgtgagctgagggtgaagttttcccggtctgccgatgcaccagcatatcagcagggacagaatcagctgtacaacgagctgaatctgggccggagagaggagtacgacgtgctggataagaggaggggaagggaccctgagatgggaggcaagccacggagaaaaacccccaggagggcctgtataatgagctgcagaaggacaagatggccgaggcctactctgagatcggcatgaagggagagaggcgccggggcaagggacacgatggcctgtatcagggcctgagcacagccaccaaggacacctacgatgccctgcatatgcaggcactgcctccaaggtga

SEQ ID NO: 248 - protein, 529 aa, Artificial Sequence
  Synthetic Construct
MALPVTALLLPLALLLHAARPQVTLKESGPVLVKPTETLTLTCTVSGFSLNNARMGVSWIRQPPGKALEWFAHIFSTDEKSFRTSLRSRLTLSKDTSKSQVVLTMTNMDPVDTATYYCARDSSNYEGYFDYWGQGILVTVSSGGGGSGGGGSGGGGSGGGGSEIVMTQSPATLSVSPGERATLSCRASQSVSNNLAWYQQKPGQAPRLLIYGASTRATGVPARFSGSDSGTEFSLTISSLQSEDFAVYFCQQYKDWPFTFGPGTKVEIKGSGGGGSCPYSNPSLCSGGGGSCPYSNPSLCSGGGGSTTTPAPRPPTPAPTIASQPLSLRPEACRPAAGGAVHTRGLDFACDIYIWAPLAGTCGVLLLSLVITLYCKRGRKKLLYIFKQPFMRPVQTTQEEDGCSCRFPEEEEGGCELRVKFSRSADAPAYQQGQNQLYNELNLGRREEYDVLDKRRGRDPEMGGKPRRKNPQEGLYNELQKDKMAEAYSEIGMKGERRRGKGHDGLYQGLSTATKDTYDALHMQALPPR

SEQ ID NO: 249 - protein, 529 aa, Artificial Sequence
  Synthetic Construct
MALPVTALLLPLALLLHAARPQVTLKESGPVLVKPTETLTLTCTVSGFSLSNARMGVSWIRQPPGKALEWLAHIFSTDEKSIRRSLRSRLTLSKDTSKSQVVLTMTNMDPVDTATYFCARDSSNYEGYFDYWGQGTLVTVSSGGGGSGGGGSGGGGSGGGGSEVVMTQSPATLSVSPGERVTLSCRASQSVSSNFAWYQQRPGQAPRLLLYGATTRATGLPGRFSGSGSGTENILTISSLQSEDFAIYFCQQYKDWPFTFGPGSKVDIKGSGGGGSCPYSNPSLCSGGGGSCPYSNPSLCSGGGGSTTTPAPRPPTPAPTIASQPLSLRPEACRPAAGGAVHTRGLDFACDIYIWAPLAGTCGVLLLSLVITLYCKRGRKKLLYIFKQPFMRPVQTTQEEDGCSCRFPEEEEGGCELRVKFSRSADAPAYQQGQNQLYNELNLGRREEYDVLDKRRGRDPEMGGKPRRKNPQEGLYNELQKDKMAEAYSEIGMKGERRRGKGHDGLYQGLSTATKDTYDALHMQALPPR

SEQ ID NO: 250 - protein, 532 aa, Artificial Sequence
  Synthetic Construct
MALPVTALLLPLALLLHAARPEVQLVESWGVLVKPGGSLRLSCAASGFIFNNAWMSWVRQAPGKGLEWIGRIKSKSDGGTTDYAAPVKDRFTISRDDSKDTLYLQMNGLKTEDTAVYFCTTAPGGPFDYWGQGTLVTVSSGGGGSGGGGSGGGGSGGGGSDIVLTQSPLSLPVTPGEPASISCRSSQSLLHRDGFNYLDWFLQKPGQSPQLLIYLASSRASGVPDRFSGSDSGTDFTLKISRVEAEDVGVYYCMQALQTPITFGQGTRLEIKGSGGGGSCPYSNPSLCSGGGGSCPYSNPSLCSGGGGSTTTPAPRPPTPAPTIASQPLSLRPEACRPAAGGAVHTRGLDFACDIYIWAPLAGTCGVLLLSLVITLYCKRGRKKLLYIFKQPFMRPVQTTQEEDGCSCRFPEEEEGGCELRVKFSRSADAPAYQQGQNQLYNELNLGRREEYDVLDKRRGRDPEMGGKPRRKNPQEGLYNELQKDKMAEAYSEIGMKGERRRGKGHDGLYQGLSTATKDTYDALHMQALPPR

SEQ ID NO: 251 - protein, 531 aa, Artificial Sequence
  Synthetic Construct
MALPVTALLLPLALLLHAARPEVQLVESGGGLVKPGGSLRLSCEASGFTFSDAWMSWVRQAPGKGLEWVGRIKSKTDGGTTDYVVPLNGRFIISRDDSRNTLYLQLNNLKTEDTAVYYCTTVPGSYGYWGQGTLVTVSSGGGGSGGGGSGGGGSGGGGSDIVMTQSPLSLPVTPGEPASISCRSSQSLLHNKRNNYLDWFLQKPGQSPQLLIYLASNRASGVPDRFSGGGSGTDFTLKISRVEAEDVGVYYCMQAQQTPITFGQGTRLEIKGSGGGGSCPYSNPSLCSGGGGSCPYSNPSLCSGGGGSTTTPAPRPPTPAPTIASQPLSLRPEACRPAAGGAVHTRGLDFACDIYIWAPLAGTCGVLLLSLVITLYCKRGRKKLLYIFKQPFMRPVQTTQEEDGCSCRFPEEEEGGCELRVKFSRSADAPAYQQGQNQLYNELNLGRREEYDVLDKRRGRDPEMGGKPRRKNPQEGLYNELQKDKMAEAYSEIGMKGERRRGKGHDGLYQGLSTATKDTYDALHMQALPPR

SEQ ID NO: 252 - DNA, 1590 bp, Artificial Sequence
  Synthetic Construct
atggcactgccagtgaccgccctgctgctgcctctggccctgctgctgcacgcagccagaccccaggtgacactgaaggagagcggccccgtgctggtgaagcctacagagacactgaccctgacctgcacagtgagcggcttctccctgaacaatgcaaggatgggcgtgtcctggatcaggcagccacctggcaaggccctggagtggttcgcccacatctttagcaccgacgagaagtcctttcgcacatctctgagaagcaggctgaccctgagcaaggatacaagcaagtcccaggtggtgctgaccatgacaaacatggaccctgtggataccgccacatactattgtgcccgggacagctccaattacgagggctatttcgattactggggccagggcatcctggtgaccgtgtctagcggcggcggcggctctggaggaggaggaagcggaggaggaggatccggcggcggcggctctgagatcgtgatgacccagtccccagccacactgtctgtgagcccaggagagagagccaccctgtcttgcagggcctcccagtctgtgagcaacaatctggcctggtatcagcagaagcctggccaggccccaaggctgctgatctacggagcaagcaccagagcaacaggagtgcctgcaaggttctccggatctgacagcggcaccgagttttctctgacaatctcctctctgcagagcgaggacttcgccgtgtatttttgtcagcagtacaaggattggccattcacctttggccccggcacaaaggtggagatcaagggctccggaggaggaggatcctgcccctattccaacccttctctgtgcagcggaggaggaggaagctgtccatactccaatccctccctgtgctccggcggcggaggatccaccacaaccccagcacctagaccaccaaccccagcaccaacaatcgcatcccagcctctgtctctgcggcccgaggcatgcaggccagcagcaggcggcgccgtgcacaccaggggcctggactttgcctgcgatatctatatctgggcaccactggcaggaacctgtggcgtgctgctgctgagcctggtcatcaccctgtattgcaagcgcggccggaagaagctgctgtacatcttcaagcagccttttatgcgcccagtgcagacaacccaggaggaggacggctgctcctgtcggttccctgaagaggaggagggaggatgtgagctgcgcgtgaagttttcccggtctgccgatgccccagcctatcagcagggccagaaccagctgtacaacgagctgaatctgggccggagagaggagtacgacgtgctggataagaggaggggaagagatcccgagatgggaggcaagcctcggagaaagaacccacaggagggcctgtataatgagctgcagaaggacaagatggccgaggcctactctgagatcggcatgaagggagagaggcgccggggcaagggacacgatggcctgtatcagggcctgtccaccgccacaaaggacacctacgatgccctgcacatgcaggccctgcctccaaggtga

SEQ ID NO: 253 - DNA, 1590 bp, Artificial Sequence
  Synthetic Construct
atggcactgccagtgaccgccctgctgctgcctctggccctgctgctgcacgcagccagaccccaggtgacactgaaggagtccggccccgtgctggtgaagcctacagagacactgaccctgacctgcacagtgagcggcttctctctgagcaacgcaaggatgggcgtgtcctggatcaggcagccacctggcaaggccctggagtggctggcccacatcttttccaccgacgagaagtctatccggagaagcctgcgctcccggctgaccctgagcaaggatacatccaagtctcaggtggtgctgaccatgacaaacatggaccctgtggataccgccacatacttctgtgcccgggacagctccaattacgagggctattttgattactggggccagggcaccctggtgacagtgtctagcggaggaggaggaagcggaggaggaggatcaggcggcggcggctctggcggcggcggcagcgaggtggtcatgacccagtctccagccacactgagcgtgtccccaggagagcgcgtgaccctgagctgccgggcctctcagagcgtgtcctctaacttcgcctggtatcagcagcggcccggacaggcaccaaggctgctgctgtacggagcaaccacaagagcaacaggcctgcctggcaggttttccggctctggcagcggcaccgagaatatcctgacaatcagctccctgcagagcgaggacttcgccatctatttttgtcagcagtacaaggattggccattcacctttggccccggctccaaggtggacatcaagggatccggaggaggaggatcttgcccctattctaaccctagcctgtgctccggaggaggaggatcctgtccatactctaatccatccctgtgcagcggaggaggaggatctaccacaaccccagcacctagaccaccaaccccagcacccacaatcgcctctcagcctctgagcctgcgcccagaggcatgcaggccagcagcaggaggagcagtgcacaccaggggcctggacttcgcctgcgatatctatatctgggcaccactggcaggaacctgtggcgtgctgctgctgtccctggtcatcaccctgtattgcaagagaggcaggaagaagctgctgtacatcttcaagcagccttttatgcgcccagtgcagacaacccaggaggaggacggctgcagctgtcggttccctgaagaggaggagggcggctgtgagctgagagtgaagttttccaggtctgccgatgccccagcctatcagcagggccagaatcagctgtacaacgagctgaatctgggcaggcgcgaggagtacgacgtgctggataagaggagaggacgcgatcccgagatgggaggcaagcctaggcgcaagaacccacaggagggcctgtataatgagctgcagaaggacaagatggccgaggcctactctgagatcggcatgaagggagagcggagaaggggcaagggacacgatggcctgtatcagggcctgagcaccgccacaaaggacacctacgatgccctgcacatgcaggccctgcctccaaggtga

SEQ ID NO: 254 - DNA, 1599 bp, Artificial Sequence
  Synthetic Construct
atggccctgccagtgaccgccctgctgctgccactggccctgctgctgcacgccgccagacctgaggtgcagctggtggagagctggggcgtgctggtgaagccaggaggctctctgaggctgagctgcgcagcatccggcttcatctttaacaatgcctggatgtcctgggtgagacaggcaccaggcaagggcctggagtggatcggcaggatcaagagcaagtccgacggaggaaccacagattacgcagcacccgtgaaggaccgcttcacaatctctcgggacgatagcaaggataccctgtatctgcagatgaacggcctgaagacagaggacaccgccgtgtacttctgcaccacagccccaggcggcccctttgattattggggccagggcacactggtgaccgtgagctccggaggaggaggaagcggcggaggaggcagcggcggcggcggctctggcggcggcggcagcgacatcgtgctgacacagagcccactgtccctgcctgtgaccccaggagagcccgcctctatcagctgtcgctctagccagagcctgctgcaccgggacggcttcaattacctggattggtttctgcagaagcctggccagagcccacagctgctgatctatctggcctcctctagagcatccggagtgcctgacaggttctccggatctgacagcggcacagacttcaccctgaagatctcccgcgtggaggcagaggatgtgggcgtgtactattgcatgcaggccctgcagacaccaatcaccttcggccagggcacacggctggagatcaagggatccggaggaggaggatcttgcccctactctaaccctagcctgtgcagcggcggaggaggatcttgtccatattctaatccaagcctgtgcagcgggggaggaggaagcaccacaacccctgcaccaagaccccctacaccagcacctaccatcgcatcccagccactgtctctgcggcccgaggcatgtaggccagcagcaggaggagcagtgcacaccaggggcctggactttgcctgcgatatctacatctgggcaccactggcaggaacatgtggcgtgctgctgctgagcctggtcatcaccctgtactgcaagagaggcaggaagaagctgctgtatatcttcaagcagccttttatgcgcccagtgcagacaacccaggaggaggacggctgctcctgtaggttcccagaagaggaggagggaggatgtgagctgcgcgtgaagttttcccggtctgccgatgcacctgcataccagcagggacagaaccagctgtataacgagctgaatctgggccggagagaggagtacgacgtgctggataagaggaggggacgcgatcctgagatgggaggcaagccccggagaaagaaccctcaggagggcctgtacaatgagctgcagaaggacaagatggccgaggcctattccgagatcggcatgaagggagagaggcgccggggcaagggacacgatggcctgtaccagggcctgtctacagccaccaaggacacctatgatgccctgcacatgcaggccctgccaccaaggtga

SEQ ID NO: 255 - DNA, 1596 bp, Artificial Sequence
  Synthetic Construct
atggcactgccagtgacagccctgctgctgcctctggccctgctgctgcacgcagccagaccagaggtgcagctggtggagtccggaggaggcctggtgaagccaggaggctccctgaggctgtcttgcgaggccagcggcttcacctttagcgacgcctggatgtcctgggtgagacaggcaccaggcaagggcctggagtgggtgggcaggatcaagagcaagacagacggcggcaccacagattacgtggtgcctctgaacggccggttcatcatctcccgcgacgattctcggaataccctgtatctgcagctgaacaatctgaagacagaggataccgccgtgtactattgcaccacagtgcctggctcctacggctattggggccagggcacactggtgaccgtgagctccggcggcggcggctctggaggaggaggaagcggaggaggaggaagcgggggcggcggctctgacatcgtgatgacacagtctccactgagcctgccagtgaccccaggagagcctgcctccatctcttgtcgctctagccagtccctgctgcacaacaagcggaacaattacctggattggttcctgcagaagccaggccagtctccccagctgctgatctatctggccagcaatagagcctccggagtgccagacaggttctctggaggaggaagcggaacagacttcaccctgaagatcagccgcgtggaggcagaggacgtgggcgtgtactattgcatgcaggcccagcagacacccatcacctttggccagggaacccggctggagatcaagggctccggaggaggaggatcctgcccttactccaacccatctctgtgcagcggaggaggaggatcttgtccatattccaatccttccctgtgctccggaggaggaggaagcaccacaacccctgcaccaagaccccctacaccagcacctaccatcgcatcccagcctctgtctctgcggcccgaggcatgtaggccagcagcaggcggcgccgtgcacaccaggggcctggactttgcctgcgatatctacatctgggcaccactggcaggaacatgtggcgtgctgctgctgtctctggtcatcaccctgtactgcaagagaggcaggaagaagctgctgtatatcttcaagcagcccttcatgcggcccgtgcagacaacccaggaggaggacggctgcagctgtcggttccctgaagaggaggagggaggatgtgagctgcgcgtgaagtttagccggtccgccgatgcaccagcataccagcagggccagaaccagctgtataacgagctgaatctgggccggagagaggagtacgacgtgctggataagaggaggggacgcgatcctgagatgggaggcaagcctcggagaaagaacccacaggagggcctgtacaatgagctgcagaaggacaagatggccgaggcctatagcgagatcggcatgaagggagagaggcgccggggcaagggacacgatggcctgtaccagggcctgtccacagccaccaaggacacctatgatgccctgcacatgcaggccctgccaccaaggtga

SEQ ID NO: 256 - protein, 9 aa, Artificial Sequence
  Synthetic Construct
CPYSNPSLC

SEQ ID NO: 257 - protein, 255 aa, Artificial Sequence
  Synthetic Construct
MALPVTALLLPLALLLHAARPDVVMTQSPLSLPVTLGQPASISCKSSQSLLYSNGKTYLNWFQQRPGQSPRRLIYQVSKLDSGVPDRFSGSGSGTDFTLKISRVEAEDVGVYYCGQDTHFPLTFGGGTKVEIKGGGGSGGGGSGGGGSGGGGSQVQLVQSGAEVKKPGASVKVSCKASGYTFTDYTLHWVRQAPGQGLEWMGGIWPITGGTTYNQKFKGRVTMTRDTSTSTVYMELSSLRSEDTAVYYCARGEAQ

SEQ ID NO: 258 - protein, 255 aa, Artificial Sequence
  Synthetic Construct
MALPVTALLLPLALLLHAARPQVTLKESGPVLLKPTETLTLTCTVSGFSLSNPRMGVSWIRQPPGKALEWFAHIFSTDEKSLKLSLRSRLTLSKDTSKSQVVLTMTNMAPVDSATYYCARDSSNYEGYFDFWGQGTLVTVSSGGGGSGGGGSGGGGSGGGGSEVVLTQSPATLSVSPGERATLSCRASQSVRSNLAWYQQKSGQAPRLLIYGSTIRATGVPARFSGSGSGTEFTLTISSLQSEDFAVYYCQQYSD

SEQ ID NO: 259 - protein, 255 aa, Artificial Sequence
  Synthetic Construct
MALPVTALLLPLALLLHAARPQVTLKESGPVLVKPTETLTLTCTVSGFSLSNARMGVSWIRQPPGKALEWLAHIFSTDEKSIRRSLRSRLTLSKDTSKSQVVLTMTNMDPVDTATYFCARDSSNYEGYFDYWGQGTLVTVSSGGGGSGGGGSGGGGSGGGGSEVVMTQSPATLSVSPGERVTLSCRASQSVSSNFAWYQQRPGQAPRLLLYGATTRATGLPGRFSGSGSGTENILTISSLQSEDFAIYFCQQYKD

SEQ ID NO: 260 - protein, 255 aa, Artificial Sequence
  Synthetic Construct
MALPVTALLLPLALLLHAARPQVTLKESGPVLVKPTETLTLTCTVSGFSLSNARMGVSWIRQPPGKALEWLGHIFSTDEKSYSTSLRGRITISKDTSRGLVVLTLTNMDPVDTATYYCARDSSNYEGYFDFWGPGFLVTVSSGGGGSGGGGSGGGGSGGGGSEIVMTQSPATLSVSPGERATLSCRVSQSIGANLAWYQQKFGQAPRLLIYGASTRATGIPVRFSGGGSGTEFTLTISSLQSEDFAIYSCQQYIY

SEQ ID NO: 261 - protein, 255 aa, Artificial Sequence
  Synthetic Construct
MALPVTALLLPLALLLHAARPQVTLKESGPVLVKPTETLTLTCTVSGFSLNNARMGVSWIRQPPGKALEWFAHIFSTDEKSFRTSLRSRLTLSKDTSKSQVVLTMTNMDPVDTATYYCARDSSNYEGYFDYWGQGILVTVSSGGGGSGGGGSGGGGSGGGGSEIVMTQSPATLSVSPGERATLSCRASQSVSNNLAWYQQKPGQAPRLLIYGASTRATGVPARFSGSDSGTEFSLTISSLQSEDFAVYFCQQYKD

SEQ ID NO: 262 - protein, 255 aa, Artificial Sequence
  Synthetic Construct
MALPVTALLLPLALLLHAARPEVNLVESGGGLVKPGGSLRLSCEASGFTFSYAWMSWVRQAPGKGLEWVGRIKSIADGGATDYAAPVRNRFTISRDDSRNTLYLEMHSLKTEDTAVYYCTTIPGNDAFDMWGQGTMVTVSSGGGGSGGGGSGGGGSGGGGSDIVLTQSPLSLSVTPGEPASISCRSSQSLLYSNGKNYLDWFLHKPGQSPQLLIYLGSNRASGVPDRFSGSGSGIDFILKISRVEAEDVGVYYCM

SEQ ID NO: 263 - protein, 255 aa, Artificial Sequence
  Synthetic Construct
MALPVTALLLPLALLLHAARPEVNLVESGGGLVKPGGSLRLSCEASGFTFSYAWMSWVRQAPGKGLEWVGRIKSITDGGVIDYAAPVRNRCTISRDDSRNTLYLEMHSLKTEDTAVYYCTTIPGNDDFDMWGQGRMVTVSSGGGGSGGGGSGGGGSGGGGSDIVLTQSPLSLSVTPGEPASISCRSSQSLLYSNGKNYLDWFLHKPGQSPQLLIYLGSNRASGVPDRFSGSGSGIDFILKISRVEAEDVGVYYCM

SEQ ID NO: 264 - protein, 255 aa, Artificial Sequence
  Synthetic Construct
MALPVTALLLPLALLLHAARPEVQLVESWGVLVKPGGSLRLSCAASGFIFNNAWMSWVRQAPGKGLEWIGRIKSKSDGGTTDYAAPVKDRFTISRDDSKDTLYLQMNGLKTEDTAVYFCTTAPGGPFDYWGQGTLVTVSSGGGGSGGGGSGGGGSGGGGSDIVLTQSPLSLPVTPGEPASISCRSSQSLLHRDGFNYLDWFLQKPGQSPQLLIYLASSRASGVPDRFSGSDSGTDFTLKISRVEAEDVGVYYCMQ

SEQ ID NO: 265 - protein, 255 aa, Artificial Sequence
  Synthetic Construct
MALPVTALLLPLALLLHAARPEVQLVESGGGLVKPGGSLRLSCEASGFTFSDAWMSWVRQAPGKGLEWVGRIKSKTDGGTTDYVVPLNGRFIISRDDSRNTLYLQLNNLKTEDTAVYYCTTVPGSYGYWGQGTLVTVSSGGGGSGGGGSGGGGSGGGGSDIVMTQSPLSLPVTPGEPASISCRSSQSLLHNKRNNYLDWFLQKPGQSPQLLIYLASNRASGVPDRFSGGGSGTDFTLKISRVEAEDVGVYYCMQA

SEQ ID NO: 266 - protein, 255 aa, Artificial Sequence
  Synthetic Construct
MALPVTALLLPLALLLHAARPQVQLVQSGAEVKKPGSSVKVSCKASGDTFSSNAISWVRQAPGQGLEWMGVIIPIFGTADYAQKFQGRVTITADESTSTAYMELSSLRSEDTAVYYCARHTYHEYAGGYYGGAMDPWGQGTLVTVSSGGGGSGGGGSGGGGSGGGGSELQSVLTQPPSASGTPGQRVTISCSGSSSNIGSNYVYWYQQLPGTAPKILIYRNNQRPSGVPDRFSGSKSGTSASLAISGLRSEDEAD

SEQ ID NO: 267 - protein, 9 aa, Artificial Sequence
  Synthetic Construct
GFTFSYAWM

SEQ ID NO: 268 - protein, 255 aa, Homo sapien
LTPQQVVAIASNGGGKQALETVQRLLPVLCQAHGLTPQQVVAIASNNGGKQALETVQRLLPVLCQAHGLTPQQVVAIASNGGGKQALETVQRLLPVLCQAHGLTPEQVVAIASHDGGKQALETVQRLLPVLCQAHGLTPEQVVAIASHDGGKQALETVQRLLPVLCQAHGLTPEQVVAIASHDGGKQALETVQRLLPVLCQAHGLTPEQVVAIASNIGGKQALETVQALLPVLCQAHGLTPEQVVAIASHDGGKQ

SEQ ID NO: 269 - protein, 255 aa, Artificial Sequence
  Synthetic Construct
LTPEQVVAIASHDGGKQALETVQRLLPVLCQAHGLTPQQVVAIASNGGGKQALETVQRLLPVLCQAHGLTPEQVVAIASHDGGKQALETVQRLLPVLCQAHGLTPEQVVAIASNIGGKQALETVQALLPVLCQAHGLTPQQVVAIASNNGGKQALETVQRLLPVLCQAHGLTPEQVVAIASHDGGKQALETVQRLLPVLCQAHGLTPQQVVAIASNGGGKQALETVQRLLPVLCQAHGLTPQQVVAIASNNGGKQ

SEQ ID NO: 270 - protein, 255 aa, Artificial Sequence
  Synthetic Construct
LTPQQVVAIASNNGGKQALETVQRLLPVLCQAHGLTPQQVVAIASNGGGKQALETVQRLLPVLCQAHGLTPQQVVAIASNNGGKQALETVQRLLPVLCQAHGLTPQQVVAIASNGGGKQALETVQRLLPVLCQAHGLTPQQVVAIASNGGGKQALETVQRLLPVLCQAHGLTPQQVVAIASNGGGKQALETVQRLLPVLCQAHGLTPQQVVAIASNNGGKQALETVQRLLPVLCQAHGLTPEQVVAIASNIGGKQ

SEQ ID NO: 271 - protein, 255 aa, Artificial Sequence
  Synthetic Construct
NPQRSTVWYLTPQQVVAIASNNGGKQALETVQRLLPVLCQAHGLTPQQVVAIASNGGGKQALETVQRLLPVLCQAHGLTPQQVVAIASNNGGKQALETVQRLLPVLCQAHGLTPQQVVAIASNNGGKQALETVQRLLPVLCQAHGLTPEQVVAIASHDGGKQALETVQRLLPVLCQAHGLTPEQVVAIASHDGGKQALETVQRLLPVLCQAHGLTPQQVVAIASNGGGKQALETVQRLLPVLCQAHGLTPQQVVA

SEQ ID NO: 272 - protein, 255 aa, Artificial Sequence
  Synthetic Construct
LTPEQVVAIASHDGGKQALETVQRLLPVLCQAHGLTPEQVVAIASHDGGKQALETVQRLLPVLCQAHGLTPEQVVAIASHDGGKQALETVQRLLPVLCQAHGLTPEQVVAIASNIGGKQALETVQALLPVLCQAHGLTPEQVVAIASHDGGKQALETVQRLLPVLCQAHGLTPEQVVAIASHDGGKQALETVQRLLPVLCQAHGLTPEQVVAIASHDGGKQALETVQRLLPVLCQAHGLTPQQVVAIASNNGGKQ

SEQ ID NO: 273 - protein, 255 aa, Artificial Sequence
  Synthetic Construct
LTPQQVVAIASNNGGKQALETVQRLLPVLCQAHGLTPQQVVAIASNNGGKQALETVQRLLPVLCQAHGLTPQQVVAIASNNGGKQALETVQRLLPVLCQAHGLTPEQVVAIASNIGGKQALETVQALLPVLCQAHGLTPQQVVAIASNNGGKQALETVQRLLPVLCQAHGLTPEQVVAIASNIGGKQALETVQALLPVLCQAHGLTPQQVVAIASNGGGKQALETVQRLLPVLCQAHGLTPEQVVAIASHDGGKQ

SEQ ID NO: 274 - protein, 255 aa, Artificial Sequence
  Synthetic Construct
LTPQQVVAIASNGGGKQALETVQRLLPVLCQAHGLTPEQVVAIASHDGGKQALETVQRLLPVLCQAHGLTPEQVVAIASHDGGKQALETVQRLLPVLCQAHGLTPQQVVAIASNGGGKQALETVQRLLPVLCQAHGLTPEQVVAIASHDGGKQALETVQRLLPVLCQAHGLTPEQVVAIASHDGGKQALETVQRLLPVLCQAHGLTPQQVVAIASNGGGKQALETVQRLLPVLCQAHGLTPEQVVAIASNIGGKQ

SEQ ID NO: 275 - protein, 255 aa, Artificial Sequence
  Synthetic Construct
LTPQQVVAIASNGGGKQALETVQRLLPVLCQAHGLTPQQVVAIASNNGGKQALETVQRLLPVLCQAHGLTPEQVVAIASHDGGKQALETVQRLLPVLCQAHGLTPQQVVAIASNGGGKQALETVQRLLPVLCQAHGLTPEQVVAIASHDGGKQALETVQRLLPVLCQAHGLTPQQVVAIASNGGGKQALETVQRLLPVLCQAHGLTPQQVVAIASNGGGKQALETVQRLLPVLCQAHGLTPEQVVAIASNIGGKQ

SEQ ID NO: 276 - protein, 136 aa, Homo sapien
CPYSNPSLCSGGGGSELPTQGTFSNVSTNVSPAKPTTTACPYSNPSLCSGGGGSPAPRPPTPAPTIASQPLSLRPEACRPAAGGAVHTRGLDFACDIYIWAPLAGTCGVLLLSLVITLYCNHRNRRRVCKCPRPVV

SEQ ID NO: 277 - DNA, 1509 bp, Artificial Sequence
  Synthetic Construct
atggctctgcccgtcaccgctctgctgctgcctctggccctgctgctgcacgcagcaaggccacaggtgcagctggtgcagtccggagcagaggtgaagaagcctggcagctccgtgaaggtgagctgcaaggcctccggcgacacattctctagcaacgcaatcagctgggtgcgccaggcccctggccagggactggagtggatgggcgtgatcatccctatcttcggcaccgccgactatgcccagaagtttcagggccgggtgacaatcaccgccgatgagtctacaagcaccgcctacatggagctgtcctctctgagatccgaggacacagccgtgtactattgtgccaggcacacctatcacgagtacgcaggaggatactatggaggagcaatggatccttggggacagggcacactggtgaccgtgagctccggcggcggcggctctggaggaggaggaagcggaggaggaggaagcgggggcggcggctctgagctgcagagcgtgctgacccagccaccttccgcctctggaacaccaggccagagggtgaccatcagctgctccggatctagctccaacatcggctccaattacgtgtattggtaccagcagctgccaggcacagcccccaagatcctgatctaccgcaacaatcagcggccttctggcgtgccagatagattctctggcagcaagtccggcacctctgccagcctggcaatctccggcctgaggtctgaggacgaggccgattactattgcgccgcctgggacgataacctgagcggctgggtgtttggcacaggcaccaagctgacagtgctgaccacaacccctgcaccaagaccaccaacaccagcacctaccatcgcaagccagccactgtccctgagacccgaggcctgtaggcctgcagcaggaggagcagtgcacaccaggggcctggactttgcctgcgatatctatatctgggcaccactggcaggaacatgtggcgtgctgctgctgagcctggtcatcaccctgtattgcaagagaggcaggaagaagctgctgtacatcttcaagcagccctttatgcgccctgtgcagacaacccaggaggaggacggctgcagctgtcggttcccagaagaggaggagggaggatgtgagctgagggtgaagttttcccggtctgccgatgcaccagcatatcagcagggacagaatcagctgtacaacgagctgaatctgggccggagagaggagtacgacgtgctggataagaggaggggaagggaccctgagatgggaggcaagccacggagaaagaacccccaggagggcctgtataatgagctgcagaaggacaagatggccgaggcctactctgagatcggcatgaagggagagaggcgccggggcaagggacacgatggcctgtatcagggcctgagcacagccaccaaggacacctacgatgccctgcatatgcaggcactgcctccaaggtga